European Patent Application EP 4 471 138 A1, published December 4, 2024. Title: TRUNCATED FORMS OF IGA PROTEASE, FUSION PROTEINS COMPRISING A TRUNCATED FORM OF IGA PROTEASE AND USES THEREOF. Applicant: Peking University First Hospital. The sequence listing filed with the application follows.

SEQUENCE LISTING (87 sequences)

SEQ ID NO: 1 - protein, 1234 aa, Clostridium ramosum
MTKKLMTKKITAIFLALYMAISVLPMTIQAASKPDIKVGDYVKMGVYNNASILWRCVSIDNNGPLMLADKIVDTLAYDAKTNDNSNSKSHSRSYKRDDYGSNYWKDSNMRSWLNSTAAEGKVDWLCGNPPKDGYVSGVGAYNEKAGFLNAFSKSEIAAMKTVTQRSLVSHPEYNKGIVDGDANSDLLYYTDISEAVANYDSSYFETTTEKVFLLDVKQANAVWKNLKGYYVAYNNDGMAWPYWLRTPVTDCNHDMRYISSSGQVGRYAPWYSDLGVRPAFYLDSEYFVTTSGSGSQSSPYIGSAPNKQEDDYTISEPAEDANPDWNVSTEQSIQLTLGPWYSNDGKYSNPTIPVYTIQKTRSDTENMVVVVCGEGYTKSQQGKFINDVKRLWQDAMKYEPYRSYADRFNVYALCTASESTFDNGGSTFFDVIVDKYNSPVISNNLHGSQWKNHIFERCIGPEFIEKIHDAHIKKKCDPNTIPSGSEYEPYYYVHDYIAQFAMVVNTKSDFGGAYNNREYGFHYFISPSDSYRASKTFAHEFGHGLLGLGDEYSNGYLLDDKELKSLNLSSVEDPEKIKWRQLLGFRNTYTCRNAYGSKMLVSSYECIMRDTNYQFCEVCRLQGFKRMSQLVKDVDLYVATPEVKEYTGAYSKPSDFTDLETSSYYNYTYNRNDRLLSGNSKSRFNTNMNGKKIELRTVIQNISDKNARQLKFKMWIKHSDGSVATDSSGNPLQTVQTFDIPVWNDKANFWPLGALDHIKSDFNSGLKSCSLIYQIPSDAQLKSGDTVAFQVLDENGNVLADDNTETQRYTTVSIQYKFEDGSEIPNTAGGTFTVPYGTKLDLTPAKTLYDYEFIKVDGLNKPIVSDGTVVTYYYKNKNEEHTHNLTLVAAKAATCTTAGNSAYYTCDGCDKWFADATGSVEITDKTSVKIPAPGHTAGTEWKSDDTNHWHECTVAGCGVIIESTKSAHTAGEWIVDTPATATTAGTKHKECTVCHRVLETQPIPSTGTELKIIAGDNQIYNKASGSDVTITCNGDFAKFTGIKVDGSVVDSSNYTAVSGSTVLTLKASYLGTLTDGSHTITFVYTDGEANANLTVRTAGSGHIHDYGTEWKSNADNHWHECNCGDKKDEAAHSFKWVVDKEATATKKGSKHEECKICGYKRSAVEIPATGTSTAPTDTTKPNDTTKPGNTNGSEKSPQTGDNSNIFLWFALLFVSAAGVTGITAYNKKKKEHAE

SEQ ID NO: 2 - protein, 1009 aa, synthetic construct
HMASKPDIKVGDYVKMGVYNNASILWRCVSIDNNGPLMLADKIVDTLAYDAKTNDNSNSKSHSRSYKRDDYGSNYWKDSNMRSWLNSTAAEGKVDWLCGNPPKDGYVSGVGAYNEKAGFLNAFSKSEIAAMKTVTQRSLVSHPEYNKGIVDGDANSDLLYYTDISEAVANYDSSYFETTTEKVFLLDVKQANAVWKNLKGYYVAYNNDGMAWPYWLRTPVTDCNHDMRYISSSGQVGRYAPWYSDLGVRPAFYLDSEYFVTTSGSGSQSSPYIGSAPNKQEDDYTISEPAEDANPDWNVSTEQSIQLTLGPWYSNDGKYSNPTIPVYTIQKTRSDTENMVVVVCGEGYTKSQQGKFINDVKRLWQDAMKYEPYRSYADRFNVYALCTASESTFDNGGSTFFDVIVDKYNSPVISNNLHGSQWKNHIFERCIGPEFIEKIHDAHIKKKCDPNTIPSGSEYEPYYYVHDYIAQFAMVVNTKSDFGGAYNNREYGFHYFISPSDSYRASKTFAHEFGHGLLGLGDEYSNGYLLDDKELKSLNLSSVEDPEKIKWRQLLGFRNTYTCRNAYGSKMLVSSYECIMRDTNYQFCEVCRLQGFKRMSQLVKDVDLYVATPEVKEYTGAYSKPSDFTDLETSSYYNYTYNRNDRLLSGNSKSRFNTNMNGKKIELRTVIQNISDKNARQLKFKMWIKHSDGSVATDSSGNPLQTVQTFDIPVWNDKANFWPLGALDHIKSDFNSGLKSCSLIYQIPSDAQLKSGDTVAFQVLGGGGSEPKSCDKTHTCPPCPAPELLGGPSVFLFPPKPKDTLMISRTPEVTCVVVDVSHEDPEVKFNWYVDGVEVHNAKTKPREEQYNSTYRVVSVLTVLHQDWLNGKEYKCKVSNKALPAPIEKTISKAKGQPREPQVYTLPPSRDELTKNQVSLTCLVKGFYPSDIAVEWESNGQPENNYKTTPPVLDSDGSFFLYSKLTVDKSRWQQGNVFSCSVMHEALHNHYTQKSLSLSPGKHHHHHHAA

SEQ ID NO: 3 - DNA, 3032 bp, synthetic construct
  source 1..3032: mol_type = other DNA
catatggcgagcaaaccggacatcaaagtgggcgactacgtgaaaatgggtgtgtataataacgcaagcatcctgtggcgctgtgtgagcatcgacaacaatggcccgctgatgctggccgataaaattgttgacacgctggcgtatgatgctaaaaccaacgacaattcgaacagcaaatctcatagtcgttcctacaaacgcgatgactacggcagcaactattggaaagatagtaatatgcgctcctggctgaactcaaccgcggccgagggtaaagtggattggctgtgcggcaatccgccgaaagacggttacgtcagcggcgtgggtgcatataatgaaaaagctggttttctgaacgcgttctcaaaatcggaaattgcagctatgaaaacggtgacccagcgtagcctggtttctcatccggaatataataaaggcattgttgatggtgacgcgaactcggatctgctgtattacaccgacatcagcgaagcagtggctaactacgatagctcttattttgaaaccacgaccgaaaaagttttcctgctggatgtcaaacaggcgaacgccgtctggaaaaatctgaaaggctattacgtggcttacaacaatgatggtatggcatggccgtattggctgcgtaccccggtgacggattgtaatcatgacatgcgctatattagttcctcaggccaggttggtcgttacgctccgtggtattctgatctgggcgtccgtccggcgttttacctggacagtgaatatttcgtgacgaccagcggctctggtagtcagtcgagcccgtacattggttccgcgccgaacaaacaagaagatgactataccatctcagaaccggcggaagatgccaacccggactggaatgtttcgacggaacagagcattcaactgaccctgggcccgtggtactcgaatgatggtaaatatagcaacccgaccattccggtgtataccatccagaaaacgcgctcggataccgaaaacatggtggttgtcgtgtgcggcgaaggttataccaaatcacagcaaggcaaatttatcaatgatgttaaacgtctgtggcaggacgctatgaaatatgaaccgtaccgtagctatgcggatcgctttaatgtgtatgcactgtgtacggcttccgaatcaaccttcgataacggcggttctacctttttcgatgtgatcgttgacaaatacaactctccggttatcagtaacaatctgcatggcagtcagtggaaaaatcacatttttgaacgctgcatcggtccggaattcattgaaaaaatccatgatgcccacattaagaaaaaatgtgacccgaacaccatcccgtcgggtagcgaatacgaaccgtattactatgtgcatgattatattgcacagtttgctatggttgtcaataccaaatccgacttcggcggtgcatataacaatcgcgaatacggctttcactatttcatctctccgagtgattcctaccgtgcctctaaaacctttgcacatgaattcggccacggtctgctgggcctgggtgatgaatactcgaatggttatctgctggatgacaaagaactgaaaagcctgaacctgtctagtgtggaagatccggaaaaaattaaatggcgtcagctgctgggctttcgcaatacgtacacctgccgtaacgcgtatggttctaaaatgctggtttcctcatacgaatgtatcatgcgcgataccaactatcaattttgcgaagtctgtcgcctgcagggcttcaaacgtatgagccaactggttaaagatgtcgacctgtatgtggccacgccggaagttaaagaatacaccggtgcatatagtaaaccgtccgattttacggacctggaaacctcgagctactacaactacacctacaaccgtaacgatcgcctgctgagtggcaactcaaaatcgcgtttcaatacgaacatgaatggcaagaaaattgaactgcgcaccgttattcagaacatcagcgataaaaacgcccgtcaactgaaattcaaaatgtggatcaaacattcagatggctcggtggcaaccgactctagtggtaacccgctgcagaccgtccaaacgtttgatattccggtgtggaacgacaaagccaatttctggccgctgggcgcactggatcacatcaaatccgactttaattcaggtctgaaaagctgctctctgatttatcagatcccgtctgatgctcaactgaaaagtggcgacaccgtggcgttccaggttctgggcggcggtggatccgagcccaaatcttgtgacaaaactcacacatgcccaccgtgcccagcacctgaactcctggggggaccgtcagtcttcctcttccccccaaaacccaaggacaccctcatgatctcccggacccctgaggtcacatgcgtggtggtggacgtgagccacgaagaccctgaggtcaagttcaactggtacgtggacggcgtggaggtgcataatgccaagacaaagccgcgggaggagcagtacaacagcacgtaccgggtggtcagcgtcctcaccgtcctgcaccaggactggctgaatggcaaggagtacaagtgcaaggtctccaacaaagccctcccagcccccatcgagaaaaccatctccaaagccaaagggcagccccgagaaccacaggtgtacaccctgcccccatcccgggatgagctgaccaagaaccaggtcagcctgacctgcctggtcaaaggcttctatcccagcgacatcgccgtggagtgggagagcaatgggcagccggagaacaactacaagaccacgcctcccgtgctggactccgacggctccttcttcctctacagcaagctcaccgtggacaagagcaggtggcagcaggggaacgtcttctcatgctccgtgatgcatgaggctctgcacaaccactacacgcagaagagcctctccctgtctccgggtaaacaccatcatcatcatcattaagcggccgc

SEQ ID NO: 4 - protein, 1032 aa, synthetic construct
KLMYRMQLLSCIALSLALVTNSGTASKPDIKVGDYVKMGVYNNASILWRCVSIDNNGPLMLADKIVDTLAYDAKTNDNSNSKSHSRSYKRDDYGSNYWKDSNMRSWLNSTAAEGKVDWLCGNPPKDGYVSGVGAYNEKAGFLNAFSKSEIAAMKTVTQRSLVSHPEYNKGIVDGDANSDLLYYTDISEAVANYDSSYFETTTEKVFLLDVKQANAVWKNLKGYYVAYNNDGMAWPYWLRTPVTDCNHDMRYISSSGQVGRYAPWYSDLGVRPAFYLDSEYFVTTSGSGSQSSPYIGSAPNKQEDDYTISEPAEDANPDWNVSTEQSIQLTLGPWYSNDGKYSNPTIPVYTIQKTRSDTENMVVVVCGEGYTKSQQGKFINDVKRLWQDAMKYEPYRSYADRFNVYALCTASESTFDNGGSTFFDVIVDKYNSPVISNNLHGSQWKNHIFERCIGPEFIEKIHDAHIKKKCDPNTIPSGSEYEPYYYVHDYIAQFAMVVNTKSDFGGAYNNREYGFHYFISPSDSYRASKTFAHEFGHGLLGLGDEYSNGYLLDDKELKSLNLSSVEDPEKIKRQLLGFRNTYTCRNAYGSKMLVSSYECIMRDTNYQFCEVCRLQGFKRMSQLVKDVDLYVATPEVKEYTGAYSKPSDFTDLETSSYYNYTYNRNDRLLSGNSKSRFNTNMNGKKIELRTVIQNISDKNARQLKFKMWIKHSDGSVATDSSGNPLQTVQTFDIPVWNDKANFWPLGALDHIKSDFNSGLKSCSLIYQIPSDAQLKSGDTVAFQVLGGGGSEPKSCDKTHTCPPCPAPELLGGPSVFLFPPKPKDTLMISRTPEVTCVVVDVSHEDPEVKFNWYVDGVEVHNAKTKPREEQYNSTYRVVSVLTVLHQDWLNGKEYKCKVSNKALPAPIEKTISKAKGQPREPQVYTLPPSRDELTKNQVSLTCLVKGFYPSDIAVEWESNGQPENNYKTTPPVLDSDGSFFLYSKLTVDKSRWQQGNVFSCSVMHEALHNHYTQKSLSLSPGKHHHHHHHHAA

SEQ ID NO: 5 - DNA, 3104 bp, synthetic construct
  source 1..3104: mol_type = other DNA
aagcttatgtatagaatgcagctgctgtcctgtattgctctgagcctggcactggttacaaacagcggtaccgcgagcaaaccggacatcaaagtgggcgactacgtgaaaatgggtgtgtataataacgcaagcatcctgtggcgctgtgtgagcatcgacaacaatggcccgctgatgctggccgataaaattgttgacacgctggcgtatgatgctaaaaccaacgacaattcgaacagcaaatctcatagtcgttcctacaaacgcgatgactacggcagcaactattggaaagatagtaatatgcgctcctggctgaactcaaccgcggccgagggtaaagtggattggctgtgcggcaatccgccgaaagacggttacgtcagcggcgtgggtgcatataatgaaaaagctggttttctgaacgcgttctcaaaatcggaaattgcagctatgaaaacggtgacccagcgtagcctggtttctcatccggaatataataaaggcattgttgatggtgacgcgaactcggatctgctgtattacaccgacatcagcgaagcagtggctaactacgatagctcttattttgaaaccacgaccgaaaaagttttcctgctggatgtcaaacaggcgaacgccgtctggaaaaatctgaaaggctattacgtggcttacaacaatgatggtatggcatggccgtattggctgcgtaccccggtgacggattgtaatcatgacatgcgctatattagttcctcaggccaggttggtcgttacgctccgtggtattctgatctgggcgtccgtccggcgttttacctggacagtgaatatttcgtgacgaccagcggctctggtagtcagtcgagcccgtacattggttccgcgccgaacaaacaagaagatgactataccatctcagaaccggcggaagatgccaacccggactggaatgtttcgacggaacagagcattcaactgaccctgggcccgtggtactcgaatgatggtaaatatagcaacccgaccattccggtgtataccatccagaaaacgcgctcggataccgaaaacatggtggttgtcgtgtgcggcgaaggttataccaaatcacagcaaggcaaatttatcaatgatgttaaacgtctgtggcaggacgctatgaaatatgaaccgtaccgtagctatgcggatcgctttaatgtgtatgcactgtgtacggcttccgaatcaaccttcgataacggcggttctacctttttcgatgtgatcgttgacaaatacaactctccggttatcagtaacaatctgcatggcagtcagtggaaaaatcacatttttgaacgctgcatcggtccggaattcattgaaaaaatccatgatgcccacattaagaaaaaatgtgacccgaacaccatcccgtcgggtagcgaatacgaaccgtattactatgtgcatgattatattgcacagtttgctatggttgtcaataccaaatccgacttcggcggtgcatataacaatcgcgaatacggctttcactatttcatctctccgagtgattcctaccgtgcctctaaaacctttgcacatgaattcggccacggtctgctgggcctgggtgatgaatactcgaatggttatctgctggatgacaaagaactgaaaagcctgaacctgtctagtgtggaagatccggaaaaaattaaatggcgtcagctgctgggctttcgcaatacgtacacctgccgtaacgcgtatggttctaaaatgctggtttcctcatacgaatgtatcatgcgcgataccaactatcaattttgcgaagtctgtcgcctgcagggcttcaaacgtatgagccaactggttaaagatgtcgacctgtatgtggccacgccggaagttaaagaatacaccggtgcatatagtaaaccgtccgattttacggacctggaaacctcgagctactacaactacacctacaaccgtaacgatcgcctgctgagtggcaactcaaaatcgcgtttcaatacgaacatgaatggcaagaaaattgaactgcgcaccgttattcagaacatcagcgataaaaacgcccgtcaactgaaattcaaaatgtggatcaaacattcagatggctcggtggcaaccgactctagtggtaacccgctgcagaccgtccaaacgtttgatattccggtgtggaacgacaaagccaatttctggccgctgggcgcactggatcacatcaaatccgactttaattcaggtctgaaaagctgctctctgatttatcagatcccgtctgatgctcaactgaaaagtggcgacaccgtggcgttccaggttctgggcggcggtggatccgaacctaagagttgcgataaaacccacacttgccctccctgtccggcccccgaactgctcggcggaccctcagtcttcctgttccccccaaagccaaaggacacattgatgatcagcaggactcctgaagtgacatgcgtggtcgtagacgtgtcacacgaggacccggaggtgaagttcaactggtacgtggacggagtggaggtgcataatgccaaaacaaagcccagagaagagcagtataacagtacctacagagtggtgtcagtgctgaccgtgcttcatcaggattggctgaacgggaaggagtacaagtgtaaggtgagtaataaggctctgcctgccccaattgagaagacaatctctaaagccaaggggcagccccgggaaccccaagtgtatacactcccaccgtcccgcgatgaactgacaaaaaaccaggtatcactcacttgtctggtaaagggcttctatccatctgacattgccgtggagtgggaatcaaacggccaacccgagaataattataagacaaccccgcccgtgctggattccgacggatcttttttcctgtatagcaaattgactgtcgacaaaagtcggtggcagcagggcaatgtgttttcttgcagcgtcatgcatgaggcgctgcacaaccactatactcagaagtcattgagcttgagccctggtaagcaccatcatcaccatcaccatcattaggcggccgc

SEQ ID NO: 6 - protein, 1010 aa, synthetic construct
HMASKPDIKVGDYVKMGVYNNASILWRCVSIDNNGPLMLADKIVDTLAYDAKTNDNSNSKSHSRSYKRDDYGSNYWKDSNMRSWLNSTAAEGKVDWLCGNPPKDGYVSGVGAYNEKAGFLNAFSKSEIAAMKTVTQRSLVSHPEYNKGIVDGDANSDLLYYTDISEAVANYDSSYFETTTEKVFLLDVKQANAVWKNLKGYYVAYNNDGMAWPYWLRTPVTDCNHDMRYISSSGQVGRYAPWYSDLGVRPAFYLDSEYFVTTSGSGSQSSPYIGSAPNKQEDDYTISEPAEDANPDWNVSTEQSIQLTLGPWYSNDGKYSNPTIPVYTIQKTRSDTENMVVVVCGEGYTKSQQGKFINDVKRLWQDAMKYEPYRSYADRFNVYALCTASESTFDNGGSTFFDVIVDKYNSPVISNNLHGSQWKNHIFERCIGPEFIEKIHDAHIKKKCDPNTIPSGSEYEPYYYVHDYIAQFAMVVNTKSDFGGAYNNREYGFHYFISPSDSYRASKTFAHEFGHGLLGLGDEYSNGYLLDDKELKSLNLSSVEDPEKIKWRQLLGFRNTYTCRNAYGSKMLVSSYECIMRDTNYQFCEVCRLQGFKRMSQLVKDVDLYVATPEVKEYTGAYSKPSDFTDLETSSYYNYTYNRNDRLLSGNSKSRFNTNMNGKKIELRTVIQNISDKNARQLKFKMWIKHSDGSVATDSSGNPLQTVQTFDIPVWNDKANFWPLGALDHIKSDFNSGLKSCSLIYQIPSDAQLKSGDTVAFQVLDENGNVGGGGSHHHHHHHHHHTCPPCPAPELLGGPSVFLFPPKPKDTLMISRTPEVTCVVVDVSHEDPEVKFNWYVDGVEVHNAKTKPREEQYNSTYRVVSVLTVLHQDWLNGKEYKCKVSNKALPAPIEKTISKAKGQPREPQVYTLPPSRDELTKNQVSLTCLVKGFYPSDIAVEWESNGQPENNYKTTPPVLDSDGSFFLYSKLTVDKSRWQQGNVFSCSVMHEALHNHYTQKSLSLSPGKAA

SEQ ID NO: 7 - DNA, 3035 bp, synthetic construct
  source 1..3035: mol_type = other DNA
catatggcgagcaaaccggacatcaaagtgggcgactacgtgaaaatgggtgtgtataataacgcaagcatcctgtggcgctgtgtgagcatcgacaacaatggcccgctgatgctggccgataaaattgttgacacgctggcgtatgatgctaaaaccaacgacaattcgaacagcaaatctcatagtcgttcctacaaacgcgatgactacggcagcaactattggaaagatagtaatatgcgctcctggctgaactcaaccgcggccgagggtaaagtggattggctgtgcggcaatccgccgaaagacggttacgtcagcggcgtgggtgcatataatgaaaaagctggttttctgaacgcgttctcaaaatcggaaattgcagctatgaaaacggtgacccagcgtagcctggtttctcatccggaatataataaaggcattgttgatggtgacgcgaactcggatctgctgtattacaccgacatcagcgaagcagtggctaactacgatagctcttattttgaaaccacgaccgaaaaagttttcctgctggatgtcaaacaggcgaacgccgtctggaaaaatctgaaaggctattacgtggcttacaacaatgatggtatggcatggccgtattggctgcgtaccccggtgacggattgtaatcatgacatgcgctatattagttcctcaggccaggttggtcgttacgctccgtggtattctgatctgggcgtccgtccggcgttttacctggacagtgaatatttcgtgacgaccagcggctctggtagtcagtcgagcccgtacattggttccgcgccgaacaaacaagaagatgactataccatctcagaaccggcggaagatgccaacccggactggaatgtttcgacggaacagagcattcaactgaccctgggcccgtggtactcgaatgatggtaaatatagcaacccgaccattccggtgtataccatccagaaaacgcgctcggataccgaaaacatggtggttgtcgtgtgcggcgaaggttataccaaatcacagcaaggcaaatttatcaatgatgttaaacgtctgtggcaggacgctatgaaatatgaaccgtaccgtagctatgcggatcgctttaatgtgtatgcactgtgtacggcttccgaatcaaccttcgataacggcggttctacctttttcgatgtgatcgttgacaaatacaactctccggttatcagtaacaatctgcatggcagtcagtggaaaaatcacatttttgaacgctgcatcggtccggaattcattgaaaaaatccatgatgcccacattaagaaaaaatgtgacccgaacaccatcccgtcgggtagcgaatacgaaccgtattactatgtgcatgattatattgcacagtttgctatggttgtcaataccaaatccgacttcggcggtgcatataacaatcgcgaatacggctttcactatttcatctctccgagtgattcctaccgtgcctctaaaacctttgcacatgaattcggccacggtctgctgggcctgggtgatgaatactcgaatggttatctgctggatgacaaagaactgaaaagcctgaacctgtctagtgtggaagatccggaaaaaattaaatggcgtcagctgctgggctttcgcaatacgtacacctgccgtaacgcgtatggttctaaaatgctggtttcctcatacgaatgtatcatgcgcgataccaactatcaattttgcgaagtctgtcgcctgcagggcttcaaacgtatgagccaactggttaaagatgtcgacctgtatgtggccacgccggaagttaaagaatacaccggtgcatatagtaaaccgtccgattttacggacctggaaacctcgagctactacaactacacctacaaccgtaacgatcgcctgctgagtggcaactcaaaatcgcgtttcaatacgaacatgaatggcaagaaaattgaactgcgcaccgttattcagaacatcagcgataaaaacgcccgtcaactgaaattcaaaatgtggatcaaacattcagatggctcggtggcaaccgactctagtggtaacccgctgcagaccgtccaaacgtttgatattccggtgtggaacgacaaagccaatttctggccgctgggcgcactggatcacatcaaatccgactttaattcaggtctgaaaagctgctctctgatttatcagatcccgtctgatgctcaactgaaaagtggcgacaccgtggcgttccaggttctggatgaaaacggtaatgtgggcggcggtggatcccaccatcatcaccaccatcatcatcaccacacatgcccaccgtgcccagcacctgaactcctggggggaccgtcagtcttcctcttccccccaaaacccaaggacaccctcatgatctcccggacccctgaggtcacatgcgtggtggtggacgtgagccacgaagaccctgaggtcaagttcaactggtacgtggacggcgtggaggtgcataatgccaagacaaagccgcgggaggagcagtacaacagcacgtaccgggtggtcagcgtcctcaccgtcctgcaccaggactggctgaatggcaaggagtacaagtgcaaggtctccaacaaagccctcccagcccccatcgagaaaaccatctccaaagccaaagggcagccccgagaaccacaggtgtacaccctgcccccatcccgggatgagctgaccaagaaccaggtcagcctgacctgcctggtcaaaggcttctatcccagcgacatcgccgtggagtgggagagcaatgggcagccggagaacaactacaagaccacgcctcccgtgctggactccgacggctccttcttcctctacagcaagctcaccgtggacaagagcaggtggcagcaggggaacgtcttctcatgctccgtgatgcatgaggctctgcacaaccactacacgcagaagagcctctccctgtctccgggtaaataagcggccgc

SEQ ID NO: 8 - protein, 1019 aa, synthetic construct
HMASKPDIKVGDYVKMGVYNNASILWRCVSIDNNGPLMLADKIVDTLAYDAKTNDNSNSKSHSRSYKRDDYGSNYWKDSNMRSWLNSTAAEGKVDWLCGNPPKDGYVSGVGAYNEKAGFLNAFSKSEIAAMKTVTQRSLVSHPEYNKGIVDGDANSDLLYYTDISEAVANYDSSYFETTTEKVFLLDVKQANAVWKNLKGYYVAYNNDGMAWPYWLRTPVTDCNHDMRYISSSGQVGRYAPWYSDLGVRPAFYLDSEYFVTTSGSGSQSSPYIGSAPNKQEDDYTISEPAEDANPDWNVSTEQSIQLTLGPWYSNDGKYSNPTIPVYTIQKTRSDTENMVVVVCGEGYTKSQQGKFINDVKRLWQDAMKYEPYRSYADRFNVYALCTASESTFDNGGSTFFDVIVDKYNSPVISNNLHGSQWKNHIFERCIGPEFIEKIHDAHIKKKCDPNTIPSGSEYEPYYYVHDYIAQFAMVVNTKSDFGGAYNNREYGFHYFISPSDSYRASKTFAHEFGHGLLGLGDEYSNGYLLDDKELKSLNLSSVEDPEKIKWRQLLGFRNTYTCRNAYGSKMLVSSYECIMRDTNYQFCEVCRLQGFKRMSQLVKDVDLYVATPEVKEYTGAYSKPSDFTDLETSSYYNYTYNRNDRLLSGNSKSRFNTNMNGKKIELRTVIQNISDKNARQLKFKMWIKHSDGSVATDSSGNPLQTVQTFDIPVWNDKANFWPLGALDHIKSDFNSGLKSCSLIYQIPSDAQLKSGDTVAFQVLDENGNVLADDNTETQGGGGSHHHHHHHHHHTCPPCPAPELLGGPSVFLFPPKPKDTLMISRTPEVTCVVVDVSHEDPEVKFNWYVDGVEVHNAKTKPREEQYNSTYRVVSVLTVLHQDWLNGKEYKCKVSNKALPAPIEKTISKAKGQPREPQVYTLPPSRDELTKNQVSLTCLVKGFYPSDIAVEWESNGQPENNYKTTPPVLDSDGSFFLYSKLTVDKSRWQQGNVFSCSVMHEALHNHYTQKSLSLSPGKAA

SEQ ID NO: 9 - DNA, 3062 bp, synthetic construct
  source 1..3062: mol_type = other DNA
catatggcgagcaaaccggacatcaaagtgggcgactacgtgaaaatgggtgtgtataataacgcaagcatcctgtggcgctgtgtgagcatcgacaacaatggcccgctgatgctggccgataaaattgttgacacgctggcgtatgatgctaaaaccaacgacaattcgaacagcaaatctcatagtcgttcctacaaacgcgatgactacggcagcaactattggaaagatagtaatatgcgctcctggctgaactcaaccgcggccgagggtaaagtggattggctgtgcggcaatccgccgaaagacggttacgtcagcggcgtgggtgcatataatgaaaaagctggttttctgaacgcgttctcaaaatcggaaattgcagctatgaaaacggtgacccagcgtagcctggtttctcatccggaatataataaaggcattgttgatggtgacgcgaactcggatctgctgtattacaccgacatcagcgaagcagtggctaactacgatagctcttattttgaaaccacgaccgaaaaagttttcctgctggatgtcaaacaggcgaacgccgtctggaaaaatctgaaaggctattacgtggcttacaacaatgatggtatggcatggccgtattggctgcgtaccccggtgacggattgtaatcatgacatgcgctatattagttcctcaggccaggttggtcgttacgctccgtggtattctgatctgggcgtccgtccggcgttttacctggacagtgaatatttcgtgacgaccagcggctctggtagtcagtcgagcccgtacattggttccgcgccgaacaaacaagaagatgactataccatctcagaaccggcggaagatgccaacccggactggaatgtttcgacggaacagagcattcaactgaccctgggcccgtggtactcgaatgatggtaaatatagcaacccgaccattccggtgtataccatccagaaaacgcgctcggataccgaaaacatggtggttgtcgtgtgcggcgaaggttataccaaatcacagcaaggcaaatttatcaatgatgttaaacgtctgtggcaggacgctatgaaatatgaaccgtaccgtagctatgcggatcgctttaatgtgtatgcactgtgtacggcttccgaatcaaccttcgataacggcggttctacctttttcgatgtgatcgttgacaaatacaactctccggttatcagtaacaatctgcatggcagtcagtggaaaaatcacatttttgaacgctgcatcggtccggaattcattgaaaaaatccatgatgcccacattaagaaaaaatgtgacccgaacaccatcccgtcgggtagcgaatacgaaccgtattactatgtgcatgattatattgcacagtttgctatggttgtcaataccaaatccgacttcggcggtgcatataacaatcgcgaatacggctttcactatttcatctctccgagtgattcctaccgtgcctctaaaacctttgcacatgaattcggccacggtctgctgggcctgggtgatgaatactcgaatggttatctgctggatgacaaagaactgaaaagcctgaacctgtctagtgtggaagatccggaaaaaattaaatggcgtcagctgctgggctttcgcaatacgtacacctgccgtaacgcgtatggttctaaaatgctggtttcctcatacgaatgtatcatgcgcgataccaactatcaattttgcgaagtctgtcgcctgcagggcttcaaacgtatgagccaactggttaaagatgtcgacctgtatgtggccacgccggaagttaaagaatacaccggtgcatatagtaaaccgtccgattttacggacctggaaacctcgagctactacaactacacctacaaccgtaacgatcgcctgctgagtggcaactcaaaatcgcgtttcaatacgaacatgaatggcaagaaaattgaactgcgcaccgttattcagaacatcagcgataaaaacgcccgtcaactgaaattcaaaatgtggatcaaacattcagatggctcggtggcaaccgactctagtggtaacccgctgcagaccgtccaaacgtttgatattccggtgtggaacgacaaagccaatttctggccgctgggcgcactggatcacatcaaatccgactttaattcaggtctgaaaagctgctctctgatttatcagatcccgtctgatgctcaactgaaaagtggcgacaccgtggcgttccaggttctggatgaaaacggtaatgtgctggcggatgacaacacggaaacccagggcggcggtggatcccaccatcatcaccaccatcatcatcaccacacatgcccaccgtgcccagcacctgaactcctggggggaccgtcagtcttcctcttccccccaaaacccaaggacaccctcatgatctcccggacccctgaggtcacatgcgtggtggtggacgtgagccacgaagaccctgaggtcaagttcaactggtacgtggacggcgtggaggtgcataatgccaagacaaagccgcgggaggagcagtacaacagcacgtaccgggtggtcagcgtcctcaccgtcctgcaccaggactggctgaatggcaaggagtacaagtgcaaggtctccaacaaagccctcccagcccccatcgagaaaaccatctccaaagccaaagggcagccccgagaaccacaggtgtacaccctgcccccatcccgggatgagctgaccaagaaccaggtcagcctgacctgcctggtcaaaggcttctatcccagcgacatcgccgtggagtgggagagcaatgggcagccggagaacaactacaagaccacgcctcccgtgctggactccgacggctccttcttcctctacagcaagctcaccgtggacaagagcaggtggcagcaggggaacgtcttctcatgctccgtgatgcatgaggctctgcacaaccactacacgcagaagagcctctccctgtctccgggtaaataagcggccgc

SEQ ID NO: 10 - protein, 1028 aa, synthetic construct
HMASKPDIKVGDYVKMGVYNNASILWRCVSIDNNGPLMLADKIVDTLAYDAKTNDNSNSKSHSRSYKRDDYGSNYWKDSNMRSWLNSTAAEGKVDWLCGNPPKDGYVSGVGAYNEKAGFLNAFSKSEIAAMKTVTQRSLVSHPEYNKGIVDGDANSDLLYYTDISEAVANYDSSYFETTTEKVFLLDVKQANAVWKNLKGYYVAYNNDGMAWPYWLRTPVTDCNHDMRYISSSGQVGRYAPWYSDLGVRPAFYLDSEYFVTTSGSGSQSSPYIGSAPNKQEDDYTISEPAEDANPDWNVSTEQSIQLTLGPWYSNDGKYSNPTIPVYTIQKTRSDTENMVVVVCGEGYTKSQQGKFINDVKRLWQDAMKYEPYRSYADRFNVYALCTASESTFDNGGSTFFDVIVDKYNSPVISNNLHGSQWKNHIFERCIGPEFIEKIHDAHIKKKCDPNTIPSGSEYEPYYYVHDYIAQFAMVVNTKSDFGGAYNNREYGFHYFISPSDSYRASKTFAHEFGHGLLGLGDEYSNGYLLDDKELKSLNLSSVEDPEKIKWRQLLGFRNTYTCRNAYGSKMLVSSYECIMRDTNYQFCEVCRLQGFKRMSQLVKDVDLYVATPEVKEYTGAYSKPSDFTDLETSSYYNYTYNRNDRLLSGNSKSRFNTNMNGKKIELRTVIQNISDKNARQLKFKMWIKHSDGSVATDSSGNPLQTVQTFDIPVWNDKANFWPLGALDHIKSDFNSGLKSCSLIYQIPSDAQLKSGDTVAFQVLDENGNVLADDNTETQRYTTVSIQYGGGGSHHHHHHHHHHTCPPCPAPELLGGPSVFLFPPKPKDTLMISRTPEVTCVVVDVSHEDPEVKFNWYVDGVEVHNAKTKPREEQYNSTYRVVSVLTVLHQDWLNGKEYKCKVSNKALPAPIEKTISKAKGQPREPQVYTLPPSRDELTKNQVSLTCLVKGFYPSDIAVEWESNGQPENNYKTTPPVLDSDGSFFLYSKLTVDKSRWQQGNVFSCSVMHEALHNHYTQKSLSLSPGKAA

SEQ ID NO: 11 - DNA, 3089 bp, synthetic construct
  source 1..3089: mol_type = other DNA
catatggcgagcaaaccggacatcaaagtgggcgactacgtgaaaatgggtgtgtataataacgcaagcatcctgtggcgctgtgtgagcatcgacaacaatggcccgctgatgctggccgataaaattgttgacacgctggcgtatgatgctaaaaccaacgacaattcgaacagcaaatctcatagtcgttcctacaaacgcgatgactacggcagcaactattggaaagatagtaatatgcgctcctggctgaactcaaccgcggccgagggtaaagtggattggctgtgcggcaatccgccgaaagacggttacgtcagcggcgtgggtgcatataatgaaaaagctggttttctgaacgcgttctcaaaatcggaaattgcagctatgaaaacggtgacccagcgtagcctggtttctcatccggaatataataaaggcattgttgatggtgacgcgaactcggatctgctgtattacaccgacatcagcgaagcagtggctaactacgatagctcttattttgaaaccacgaccgaaaaagttttcctgctggatgtcaaacaggcgaacgccgtctggaaaaatctgaaaggctattacgtggcttacaacaatgatggtatggcatggccgtattggctgcgtaccccggtgacggattgtaatcatgacatgcgctatattagttcctcaggccaggttggtcgttacgctccgtggtattctgatctgggcgtccgtccggcgttttacctggacagtgaatatttcgtgacgaccagcggctctggtagtcagtcgagcccgtacattggttccgcgccgaacaaacaagaagatgactataccatctcagaaccggcggaagatgccaacccggactggaatgtttcgacggaacagagcattcaactgaccctgggcccgtggtactcgaatgatggtaaatatagcaacccgaccattccggtgtataccatccagaaaacgcgctcggataccgaaaacatggtggttgtcgtgtgcggcgaaggttataccaaatcacagcaaggcaaatttatcaatgatgttaaacgtctgtggcaggacgctatgaaatatgaaccgtaccgtagctatgcggatcgctttaatgtgtatgcactgtgtacggcttccgaatcaaccttcgataacggcggttctacctttttcgatgtgatcgttgacaaatacaactctccggttatcagtaacaatctgcatggcagtcagtggaaaaatcacatttttgaacgctgcatcggtccggaattcattgaaaaaatccatgatgcccacattaagaaaaaatgtgacccgaacaccatcccgtcgggtagcgaatacgaaccgtattactatgtgcatgattatattgcacagtttgctatggttgtcaataccaaatccgacttcggcggtgcatataacaatcgcgaatacggctttcactatttcatctctccgagtgattcctaccgtgcctctaaaacctttgcacatgaattcggccacggtctgctgggcctgggtgatgaatactcgaatggttatctgctggatgacaaagaactgaaaagcctgaacctgtctagtgtggaagatccggaaaaaattaaatggcgtcagctgctgggctttcgcaatacgtacacctgccgtaacgcgtatggttctaaaatgctggtttcctcatacgaatgtatcatgcgcgataccaactatcaattttgcgaagtctgtcgcctgcagggcttcaaacgtatgagccaactggttaaagatgtcgacctgtatgtggccacgccggaagttaaagaatacaccggtgcatatagtaaaccgtccgattttacggacctggaaacctcgagctactacaactacacctacaaccgtaacgatcgcctgctgagtggcaactcaaaatcgcgtttcaatacgaacatgaatggcaagaaaattgaactgcgcaccgttattcagaacatcagcgataaaaacgcccgtcaactgaaattcaaaatgtggatcaaacattcagatggctcggtggcaaccgactctagtggtaacccgctgcagaccgtccaaacgtttgatattccggtgtggaacgacaaagccaatttctggccgctgggcgcactggatcacatcaaatccgactttaattcaggtctgaaaagctgctctctgatttatcagatcccgtctgatgctcaactgaaaagtggcgacaccgtggcgttccaggttctggatgaaaacggtaatgtgctggcggatgacaacacggaaacccagcgctacacgaccgtttctatccaatacggcggcggtggatcccaccatcatcaccaccatcatcatcaccacacatgcccaccgtgcccagcacctgaactcctggggggaccgtcagtcttcctcttccccccaaaacccaaggacaccctcatgatctcccggacccctgaggtcacatgcgtggtggtggacgtgagccacgaagaccctgaggtcaagttcaactggtacgtggacggcgtggaggtgcataatgccaagacaaagccgcgggaggagcagtacaacagcacgtaccgggtggtcagcgtcctcaccgtcctgcaccaggactggctgaatggcaaggagtacaagtgcaaggtctccaacaaagccctcccagcccccatcgagaaaaccatctccaaagccaaagggcagccccgagaaccacaggtgtacaccctgcccccatcccgggatgagctgaccaagaaccaggtcagcctgacctgcctggtcaaaggcttctatcccagcgacatcgccgtggagtgggagagcaatgggcagccggagaacaactacaagaccacgcctcccgtgctggactccgacggctccttcttcctctacagcaagctcaccgtggacaagagcaggtggcagcaggggaacgtcttctcatgctccgtgatgcatgaggctctgcacaaccactacacgcagaagagcctctccctgtctccgggtaaataagcggccgc

SEQ ID NO: 12 - protein, 1045 aa, synthetic construct
HMASKPDIKVGDYVKMGVYNNASILWRCVSIDNNGPLMLADKIVDTLAYDAKTNDNSNSKSHSRSYKRDDYGSNYWKDSNMRSWLNSTAAEGKVDWLCGNPPKDGYVSGVGAYNEKAGFLNAFSKSEIAAMKTVTQRSLVSHPEYNKGIVDGDANSDLLYYTDISEAVANYDSSYFETTTEKVFLLDVKQANAVWKNLKGYYVAYNNDGMAWPYWLRTPVTDCNHDMRYISSSGQVGRYAPWYSDLGVRPAFYLDSEYFVTTSGSGSQSSPYIGSAPNKQEDDYTISEPAEDANPDWNVSTEQSIQLTLGPWYSNDGKYSNPTIPVYTIQKTRSDTENMVVVVCGEGYTKSQQGKFINDVKRLWQDAMKYEPYRSYADRFNVYALCTASESTFDNGGSTFFDVIVDKYNSPVISNNLHGSQWKNHIFERCIGPEFIEKIHDAHIKKKCDPNTIPSGSEYEPYYYVHDYIAQFAMVVNTKSDFGGAYNNREYGFHYFISPSDSYRASKTFAHEFGHGLLGLGDEYSNGYLLDDKELKSLNLSSVEDPEKIKWRQLLGFRNTYTCRNAYGSKMLVSSYECIMRDTNYQFCEVCRLQGFKRMSQLVKDVDLYVATPEVKEYTGAYSKPSDFTDLETSSYYNYTYNRNDRLLSGNSKSRFNTNMNGKKIELRTVIQNISDKNARQLKFKMWIKHSDGSVATDSSGNPLQTVQTFDIPVWNDKANFWPLGALDHIKSDFNSGLKSCSLIYQIPSDAQLKSGDTVAFQVLDENGNVLADDNTETQRYTTVSIQYKFEDGSEIPNTAGGTFTGGGGSHHHHHHHHHHTCPPCPAPELLGGPSVFLFPPKPKDTLMISRTPEVTCVVVDVSHEDPEVKFNWYVDGVEVHNAKTKPREEQYNSTYRVVSVLTVLHQDWLNGKEYKCKVSNKALPAPIEKTISKAKGQPREPQVYTLPPSRDELTKNQVSLTCLVKGFYPSDIAVEWESNGQPENNYKTTPPVLDSDGSFFLYSKLTVDKSRWQQGNVFSCSVMHEALHNHYTQKSLSLSPGKAA

SEQ ID NO: 13 - DNA, 3140 bp, synthetic construct
  source 1..3140: mol_type = other DNA
catatggcgagcaaaccggacatcaaagtgggcgactacgtgaaaatgggtgtgtataataacgcaagcatcctgtggcgctgtgtgagcatcgacaacaatggcccgctgatgctggccgataaaattgttgacacgctggcgtatgatgctaaaaccaacgacaattcgaacagcaaatctcatagtcgttcctacaaacgcgatgactacggcagcaactattggaaagatagtaatatgcgctcctggctgaactcaaccgcggccgagggtaaagtggattggctgtgcggcaatccgccgaaagacggttacgtcagcggcgtgggtgcatataatgaaaaagctggttttctgaacgcgttctcaaaatcggaaattgcagctatgaaaacggtgacccagcgtagcctggtttctcatccggaatataataaaggcattgttgatggtgacgcgaactcggatctgctgtattacaccgacatcagcgaagcagtggctaactacgatagctcttattttgaaaccacgaccgaaaaagttttcctgctggatgtcaaacaggcgaacgccgtctggaaaaatctgaaaggctattacgtggcttacaacaatgatggtatggcatggccgtattggctgcgtaccccggtgacggattgtaatcatgacatgcgctatattagttcctcaggccaggttggtcgttacgctccgtggtattctgatctgggcgtccgtccggcgttttacctggacagtgaatatttcgtgacgaccagcggctctggtagtcagtcgagcccgtacattggttccgcgccgaacaaacaagaagatgactataccatctcagaaccggcggaagatgccaacccggactggaatgtttcgacggaacagagcattcaactgaccctgggcccgtggtactcgaatgatggtaaatatagcaacccgaccattccggtgtataccatccagaaaacgcgctcggataccgaaaacatggtggttgtcgtgtgcggcgaaggttataccaaatcacagcaaggcaaatttatcaatgatgttaaacgtctgtggcaggacgctatgaaatatgaaccgtaccgtagctatgcggatcgctttaatgtgtatgcactgtgtacggcttccgaatcaaccttcgataacggcggttctacctttttcgatgtgatcgttgacaaatacaactctccggttatcagtaacaatctgcatggcagtcagtggaaaaatcacatttttgaacgctgcatcggtccggaattcattgaaaaaatccatgatgcccacattaagaaaaaatgtgacccgaacaccatcccgtcgggtagcgaatacgaaccgtattactatgtgcatgattatattgcacagtttgctatggttgtcaataccaaatccgacttcggcggtgcatataacaatcgcgaatacggctttcactatttcatctctccgagtgattcctaccgtgcctctaaaacctttgcacatgaattcggccacggtctgctgggcctgggtgatgaatactcgaatggttatctgctggatgacaaagaactgaaaagcctgaacctgtctagtgtggaagatccggaaaaaattaaatggcgtcagctgctgggctttcgcaatacgtacacctgccgtaacgcgtatggttctaaaatgctggtttcctcatacgaatgtatcatgcgcgataccaactatcaattttgcgaagtctgtcgcctgcagggcttcaaacgtatgagccaactggttaaagatgtcgacctgtatgtggccacgccggaagttaaagaatacaccggtgcatatagtaaaccgtccgattttacggacctggaaacctcgagctactacaactacacctacaaccgtaacgatcgcctgctgagtggcaactcaaaatcgcgtttcaatacgaacatgaatggcaagaaaattgaactgcgcaccgttattcagaacatcagcgataaaaacgcccgtcaactgaaattcaaaatgtggatcaaacattcagatggctcggtggcaaccgactctagtggtaacccgctgcagaccgtccaaacgtttgatattccggtgtggaacgacaaagccaatttctggccgctgggcgcactggatcacatcaaatccgactttaattcaggtctgaaaagctgctctctgatttatcagatcccgtctgatgctcaactgaaaagtggcgacaccgtggcgttccaggttctggatgaaaacggtaatgtgctggcggatgacaacacggaaacccagcgctacacgaccgtttctatccaatacaaattcgaagatggcagtgaaatcccgaatacggcgggcggtaccttcaccggcggcggtggatcccaccatcatcaccaccatcatcatcaccacacatgcccaccgtgcccagcacctgaactcctggggggaccgtcagtcttcctcttccccccaaaacccaaggacaccctcatgatctcccggacccctgaggtcacatgcgtggtggtggacgtgagccacgaagaccctgaggtcaagttcaactggtacgtggacggcgtggaggtgcataatgccaagacaaagccgcgggaggagcagtacaacagcacgtaccgggtggtcagcgtcctcaccgtcctgcaccaggactggctgaatggcaaggagtacaagtgcaaggtctccaacaaagccctcccagcccccatcgagaaaaccatctccaaagccaaagggcagccccgagaaccacaggtgtacaccctgcccccatcccgggatgagctgaccaagaaccaggtcagcctgacctgcctggtcaaaggcttctatcccagcgacatcgccgtggagtgggagagcaatgggcagccggagaacaactacaagaccacgcctcccgtgctggactccgacggctccttcttcctctacagcaagctcaccgtggacaagagcaggtggcagcaggggaacgtcttctcatgctccgtgatgcatgaggctctgcacaaccactacacgcagaagagcctctccctgtctccgggtaaataagcggccgc

SEQ ID NO: 14 - protein, 760 aa, synthetic construct
ASKPDIKVGDYVKMGVYNNASILWRCVSIDNNGPLMLADKIVDTLAYDAKTNDNSNSKSHSRSYKRDDYGSNYWKDSNMRSWLNSTAAEGKVDWLCGNPPKDGYVSGVGAYNEKAGFLNAFSKSEIAAMKTVTQRSLVSHPEYNKGIVDGDANSDLLYYTDISEAVANYDSSYFETTTEKVFLLDVKQANAVWKNLKGYYVAYNNDGMAWPYWLRTPVTDCNHDMRYISSSGQVGRYAPWYSDLGVRPAFYLDSEYFVTTSGSGSQSSPYIGSAPNKQEDDYTISEPAEDANPDWNVSTEQSIQLTLGPWYSNDGKYSNPTIPVYTIQKTRSDTENMVVVVCGEGYTKSQQGKFINDVKRLWQDAMKYEPYRSYADRFNVYALCTASESTFDNGGSTFFDVIVDKYNSPVISNNLHGSQWKNHIFERCIGPEFIEKIHDAHIKKKCDPNTIPSGSEYEPYYYVHDYIAQFAMVVNTKSDFGGAYNNREYGFHYFISPSDSYRASKTFAHEFGHGLLGLGDEYSNGYLLDDKELKSLNLSSVEDPEKIKWRQLLGFRNTYTCRNAYGSKMLVSSYECIMRDTNYQFCEVCRLQGFKRMSQLVKDVDLYVATPEVKEYTGAYSKPSDFTDLETSSYYNYTYNRNDRLLSGNSKSRFNTNMNGKKIELRTVIQNISDKNARQLKFKMWIKHSDGSVATDSSGNPLQTVQTFDIPVWNDKANFWPLGALDHIKSDFNSGLKSCSLIYQIPSDAQLKSGDTVAFQ

SEQ ID NO: 15 - protein, 761 aa, synthetic construct
ASKPDIKVGDYVKMGVYNNASILWRCVSIDNNGPLMLADKIVDTLAYDAKTNDNSNSKSHSRSYKRDDYGSNYWKDSNMRSWLNSTAAEGKVDWLCGNPPKDGYVSGVGAYNEKAGFLNAFSKSEIAAMKTVTQRSLVSHPEYNKGIVDGDANSDLLYYTDISEAVANYDSSYFETTTEKVFLLDVKQANAVWKNLKGYYVAYNNDGMAWPYWLRTPVTDCNHDMRYISSSGQVGRYAPWYSDLGVRPAFYLDSEYFVTTSGSGSQSSPYIGSAPNKQEDDYTISEPAEDANPDWNVSTEQSIQLTLGPWYSNDGKYSNPTIPVYTIQKTRSDTENMVVVVCGEGYTKSQQGKFINDVKRLWQDAMKYEPYRSYADRFNVYALCTASESTFDNGGSTFFDVIVDKYNSPVISNNLHGSQWKNHIFERCIGPEFIEKIHDAHIKKKCDPNTIPSGSEYEPYYYVHDYIAQFAMVVNTKSDFGGAYNNREYGFHYFISPSDSYRASKTFAHEFGHGLLGLGDEYSNGYLLDDKELKSLNLSSVEDPEKIKWRQLLGFRNTYTCRNAYGSKMLVSSYECIMRDTNYQFCEVCRLQGFKRMSQLVKDVDLYVATPEVKEYTGAYSKPSDFTDLETSSYYNYTYNRNDRLLSGNSKSRFNTNMNGKKIELRTVIQNISDKNARQLKFKMWIKHSDGSVATDSSGNPLQTVQTFDIPVWNDKANFWPLGALDHIKSDFNSGLKSCSLIYQIPSDAQLKSGDTVAFQV

SEQ ID NO: 16 - protein, 762 aa, synthetic construct
ASKPDIKVGDYVKMGVYNNASILWRCVSIDNNGPLMLADKIVDTLAYDAKTNDNSNSKSHSRSYKRDDYGSNYWKDSNMRSWLNSTAAEGKVDWLCGNPPKDGYVSGVGAYNEKAGFLNAFSKSEIAAMKTVTQRSLVSHPEYNKGIVDGDANSDLLYYTDISEAVANYDSSYFETTTEKVFLLDVKQANAVWKNLKGYYVAYNNDGMAWPYWLRTPVTDCNHDMRYISSSGQVGRYAPWYSDLGVRPAFYLDSEYFVTTSGSGSQSSPYIGSAPNKQEDDYTISEPAEDANPDWNVSTEQSIQLTLGPWYSNDGKYSNPTIPVYTIQKTRSDTENMVVVVCGEGYTKSQQGKFINDVKRLWQDAMKYEPYRSYADRFNVYALCTASESTFDNGGSTFFDVIVDKYNSPVISNNLHGSQWKNHIFERCIGPEFIEKIHDAHIKKKCDPNTIPSGSEYEPYYYVHDYIAQFAMVVNTKSDFGGAYNNREYGFHYFISPSDSYRASKTFAHEFGHGLLGLGDEYSNGYLLDDKELKSLNLSSVEDPEKIKWRQLLGFRNTYTCRNAYGSKMLVSSYECIMRDTNYQFCEVCRLQGFKRMSQLVKDVDLYVATPEVKEYTGAYSKPSDFTDLETSSYYNYTYNRNDRLLSGNSKSRFNTNMNGKKIELRTVIQNISDKNARQLKFKMWIKHSDGSVATDSSGNPLQTVQTFDIPVWNDKANFWPLGALDHIKSDFNSGLKSCSLIYQIPSDAQLKSGDTVAFQVL

SEQ ID NO: 17 - protein, 768 aa, synthetic construct
ASKPDIKVGDYVKMGVYNNASILWRCVSIDNNGPLMLADKIVDTLAYDAKTNDNSNSKSHSRSYKRDDYGSNYWKDSNMRSWLNSTAAEGKVDWLCGNPPKDGYVSGVGAYNEKAGFLNAFSKSEIAAMKTVTQRSLVSHPEYNKGIVDGDANSDLLYYTDISEAVANYDSSYFETTTEKVFLLDVKQANAVWKNLKGYYVAYNNDGMAWPYWLRTPVTDCNHDMRYISSSGQVGRYAPWYSDLGVRPAFYLDSEYFVTTSGSGSQSSPYIGSAPNKQEDDYTISEPAEDANPDWNVSTEQSIQLTLGPWYSNDGKYSNPTIPVYTIQKTRSDTENMVVVVCGEGYTKSQQGKFINDVKRLWQDAMKYEPYRSYADRFNVYALCTASESTFDNGGSTFFDVIVDKYNSPVISNNLHGSQWKNHIFERCIGPEFIEKIHDAHIKKKCDPNTIPSGSEYEPYYYVHDYIAQFAMVVNTKSDFGGAYNNREYGFHYFISPSDSYRASKTFAHEFGHGLLGLGDEYSNGYLLDDKELKSLNLSSVEDPEKIKWRQLLGFRNTYTCRNAYGSKMLVSSYECIMRDTNYQFCEVCRLQGFKRMSQLVKDVDLYVATPEVKEYTGAYSKPSDFTDLETSSYYNYTYNRNDRLLSGNSKSRFNTNMNGKKIELRTVIQNISDKNARQLKFKMWIKHSDGSVATDSSGNPLQTVQTFDIPVWNDKANFWPLGALDHIKSDFNSGLKSCSLIYQIPSDAQLKSGDTVAFQVLDENGNV

SEQ ID NO: 18 - protein, 777 aa, synthetic construct
ASKPDIKVGDYVKMGVYNNASILWRCVSIDNNGPLMLADKIVDTLAYDAKTNDNSNSKSHSRSYKRDDYGSNYWKDSNMRSWLNSTAAEGKVDWLCGNPPKDGYVSGVGAYNEKAGFLNAFSKSEIAAMKTVTQRSLVSHPEYNKGIVDGDANSDLLYYTDISEAVANYDSSYFETTTEKVFLLDVKQANAVWKNLKGYYVAYNNDGMAWPYWLRTPVTDCNHDMRYISSSGQVGRYAPWYSDLGVRPAFYLDSEYFVTTSGSGSQSSPYIGSAPNKQEDDYTISEPAEDANPDWNVSTEQSIQLTLGPWYSNDGKYSNPTIPVYTIQKTRSDTENMVVVVCGEGYTKSQQGKFINDVKRLWQDAMKYEPYRSYADRFNVYALCTASESTFDNGGSTFFDVIVDKYNSPVISNNLHGSQWKNHIFERCIGPEFIEKIHDAHIKKKCDPNTIPSGSEYEPYYYVHDYIAQFAMVVNTKSDFGGAYNNREYGFHYFISPSDSYRASKTFAHEFGHGLLGLGDEYSNGYLLDDKELKSLNLSSVEDPEKIKWRQLLGFRNTYTCRNAYGSKMLVSSYECIMRDTNYQFCEVCRLQGFKRMSQLVKDVDLYVATPEVKEYTGAYSKPSDFTDLETSSYYNYTYNRNDRLLSGNSKSRFNTNMNGKKIELRTVIQNISDKNARQLKFKMWIKHSDGSVATDSSGNPLQTVQTFDIPVWNDKANFWPLGALDHIKSDFNSGLKSCSLIYQIPSDAQLKSGDTVAFQVLDENGNVLADDNTETQ

SEQ ID NO: 19 - protein, 786 aa, synthetic construct
ASKPDIKVGDYVKMGVYNNASILWRCVSIDNNGPLMLADKIVDTLAYDAKTNDNSNSKSHSRSYKRDDYGSNYWKDSNMRSWLNSTAAEGKVDWLCGNPPKDGYVSGVGAYNEKAGFLNAFSKSEIAAMKTVTQRSLVSHPEYNKGIVDGDANSDLLYYTDISEAVANYDSSYFETTTEKVFLLDVKQANAVWKNLKGYYVAYNNDGMAWPYWLRTPVTDCNHDMRYISSSGQVGRYAPWYSDLGVRPAFYLDSEYFVTTSGSGSQSSPYIGSAPNKQEDDYTISEPAEDANPDWNVSTEQSIQLTLGPWYSNDGKYSNPTIPVYTIQKTRSDTENMVVVVCGEGYTKSQQGKFINDVKRLWQDAMKYEPYRSYADRFNVYALCTASESTFDNGGSTFFDVIVDKYNSPVISNNLHGSQWKNHIFERCIGPEFIEKIHDAHIKKKCDPNTIPSGSEYEPYYYVHDYIAQFAMVVNTKSDFGGAYNNREYGFHYFISPSDSYRASKTFAHEFGHGLLGLGDEYSNGYLLDDKELKSLNLSSVEDPEKIKWRQLLGFRNTYTCRNAYGSKMLVSSYECIMRDTNYQFCEVCRLQGFKRMSQLVKDVDLYVATPEVKEYTGAYSKPSDFTDLETSSYYNYTYNRNDRLLSGNSKSRFNTNMNGKKIELRTVIQNISDKNARQLKFKMWIKHSDGSVATDSSGNPLQTVQTFDIPVWNDKANFWPLGALDHIKSDFNSGLKSCSLIYQIPSDAQLKSGDTVAFQVLDENGNVLADDNTETQRYTTVSIQY

SEQ ID NO: 20 - protein, 803 aa, synthetic construct
ASKPDIKVGDYVKMGVYNNASILWRCVSIDNNGPLMLADKIVDTLAYDAKTNDNSNSKSHSRSYKRDDYGSNYWKDSNMRSWLNSTAAEGKVDWLCGNPPKDGYVSGVGAYNEKAGFLNAFSKSEIAAMKTVTQRSLVSHPEYNKGIVDGDANSDLLYYTDISEAVANYDSSYFETTTEKVFLLDVKQANAVWKNLKGYYVAYNNDGMAWPYWLRTPVTDCNHDMRYISSSGQVGRYAPWYSDLGVRPAFYLDSEYFVTTSGSGSQSSPYIGSAPNKQEDDYTISEPAEDANPDWNVSTEQSIQLTLGPWYSNDGKYSNPTIPVYTIQKTRSDTENMVVVVCGEGYTKSQQGKFINDVKRLWQDAMKYEPYRSYADRFNVYALCTASESTFDNGGSTFFDVIVDKYNSPVISNNLHGSQWKNHIFERCIGPEFIEKIHDAHIKKKCDPNTIPSGSEYEPYYYVHDYIAQFAMVVNTKSDFGGAYNNREYGFHYFISPSDSYRASKTFAHEFGHGLLGLGDEYSNGYLLDDKELKSLNLSSVEDPEKIKWRQLLGFRNTYTCRNAYGSKMLVSSYECIMRDTNYQFCEVCRLQGFKRMSQLVKDVDLYVATPEVKEYTGAYSKPSDFTDLETSSYYNYTYNRNDRLLSGNSKSRFNTNMNGKKIELRTVIQNISDKNARQLKFKMWIKHSDGSVATDSSGNPLQTVQTFDIPVWNDKANFWPLGALDHIKSDFNSGLKSCSLIYQIPSDAQLKSGDTVAFQVLDENGNVLADDNTETQRYTTVSIQYKFEDGSEIPNTAGGTFT

SEQ ID NO: 21 - protein, 4 aa, synthetic construct
GGGS

SEQ ID NO: 22 - protein, 5 aa, synthetic construct
GGGGS

SEQ ID NO: 23 - protein, 15 aa, synthetic construct
GGCGGCGGTGGATCC

SEQ ID NO: 24 - protein, 232 aa, synthetic construct
EPKSCDKTHTCPPCPAPELLGGPSVFLFPPKPKDTLMISRTPEVTCVVVDVSHEDPEVKFNWYVDGVEVHNAKTKPREEQYNSTYRVVSVLTVLHQDWLNGKEYKCKVSNKALPAPIEKTISKAKGQPREPQVYTLPPSRDELTKNQVSLTCLVKGFYPSDIAVEWESNGQPENNYKTTPPVLDSDGSFFLYSKLTVDKSRWQQGNVFSCSVMHEALHNHYTQKSLSLSPGK

SEQ ID NO: 25 - protein, 223 aa, synthetic construct
TCPPCPAPELLGGPSVFLFPPKPKDTLMISRTPEVTCVVVDVSHEDPEVKFNWYVDGVEVHNAKTKPREEQYNSTYRVVSVLTVLHQDWLNGKEYKCKVSNKALPAPIEKTISKAKGQPREPQVYTLPPSRDELTKNQVSLTCLVKGFYPSDIAVEWESNGQPENNYKTTPPVLDSDGSFFLYSKLTVDKSRWQQGNVFSCSVMHEALHNHYTQKSLSLSPGK

SEQ ID NO: 26 - protein, 999 aa, synthetic construct
ASKPDIKVGDYVKMGVYNNASILWRCVSIDNNGPLMLADKIVDTLAYDAKTNDNSNSKSHSRSYKRDDYGSNYWKDSNMRSWLNSTAAEGKVDWLCGNPPKDGYVSGVGAYNEKAGFLNAFSKSEIAAMKTVTQRSLVSHPEYNKGIVDGDANSDLLYYTDISEAVANYDSSYFETTTEKVFLLDVKQANAVWKNLKGYYVAYNNDGMAWPYWLRTPVTDCNHDMRYISSSGQVGRYAPWYSDLGVRPAFYLDSEYFVTTSGSGSQSSPYIGSAPNKQEDDYTISEPAEDANPDWNVSTEQSIQLTLGPWYSNDGKYSNPTIPVYTIQKTRSDTENMVVVVCGEGYTKSQQGKFINDVKRLWQDAMKYEPYRSYADRFNVYALCTASESTFDNGGSTFFDVIVDKYNSPVISNNLHGSQWKNHIFERCIGPEFIEKIHDAHIKKKCDPNTIPSGSEYEPYYYVHDYIAQFAMVVNTKSDFGGAYNNREYGFHYFISPSDSYRASKTFAHEFGHGLLGLGDEYSNGYLLDDKELKSLNLSSVEDPEKIKWRQLLGFRNTYTCRNAYGSKMLVSSYECIMRDTNYQFCEVCRLQGFKRMSQLVKDVDLYVATPEVKEYTGAYSKPSDFTDLETSSYYNYTYNRNDRLLSGNSKSRFNTNMNGKKIELRTVIQNISDKNARQLKFKMWIKHSDGSVATDSSGNPLQTVQTFDIPVWNDKANFWPLGALDHIKSDFNSGLKSCSLIYQIPSDAQLKSGDTVAFQVLGGGGSEPKSCDKTHTCPPCPAPELLGGPSVFLFPPKPKDTLMISRTPEVTCVVVDVSHEDPEVKFNWYVDGVEVHNAKTKPREEQYNSTYRVVSVLTVLHQDWLNGKEYKCKVSNKALPAPIEKTISKAKGQPREPQVYTLPPSRDELTKNQVSLTCLVKGFYPSDIAVEWESNGQPENNYKTTPPVLDSDGSFFLYSKLTVDKSRWQQGNVFSCSVMHEALHNHYTQKSLSLSPGK

SEQ ID NO: 27 - protein, 1020 aa, synthetic construct
MYRMQLLSCIALSLALVTNSGTASKPDIKVGDYVKMGVYNNASILWRCVSIDNNGPLMLADKIVDTLAYDAKTNDNSNSKSHSRSYKRDDYGSNYWKDSNMRSWLNSTAAEGKVDWLCGNPPKDGYVSGVGAYNEKAGFLNAFSKSEIAAMKTVTQRSLVSHPEYNKGIVDGDANSDLLYYTDISEAVANYDSSYFETTTEKVFLLDVKQANAVWKNLKGYYVAYNNDGMAWPYWLRTPVTDCNHDMRYISSSGQVGRYAPWYSDLGVRPAFYLDSEYFVTTSGSGSQSSPYIGSAPNKQEDDYTISEPAEDANPDWNVSTEQSIQLTLGPWYSNDGKYSNPTIPVYTIQKTRSDTENMVVVVCGEGYTKSQQGKFINDVKRLWQDAMKYEPYRSYADRFNVYALCTASESTFDNGGSTFFDVIVDKYNSPVISNNLHGSQWKNHIFERCIGPEFIEKIHDAHIKKKCDPNTIPSGSEYEPYYYVHDYIAQFAMVVNTKSDFGGAYNNREYGFHYFISPSDSYRASKTFAHEFGHGLLGLGDEYSNGYLLDDKELKSLNLSSVEDPEKIKRQLLGFRNTYTCRNAYGSKMLVSSYECIMRDTNYQFCEVCRLQGFKRMSQLVKDVDLYVATPEVKEYTGAYSKPSDFTDLETSSYYNYTYNRNDRLLSGNSKSRFNTNMNGKKIELRTVIQNISDKNARQLKFKMWIKHSDGSVATDSSGNPLQTVQTFDIPVWNDKANFWPLGALDHIKSDFNSGLKSCSLIYQIPSDAQLKSGDTVAFQVLGGGGSEPKSCDKTHTCPPCPAPELLGGPSVFLFPPKPKDTLMISRTPEVTCVVVDVSHEDPEVKFNWYVDGVEVHNAKTKPREEQYNSTYRVVSVLTVLHQDWLNGKEYKCKVSNKALPAPIEKTISKAKGQPREPQVYTLPPSRDELTKNQVSLTCLVKGFYPSDIAVEWESNGQPENNYKTTPPVLDSDGSFFLYSKLTVDKSRWQQGNVFSCSVMHEALHNHYTQKSLSLSPGK

SEQ ID NO: 28 - protein, 1006 aa, synthetic construct
ASKPDIKVGDYVKMGVYNNASILWRCVSIDNNGPLMLADKIVDTLAYDAKTNDNSNSKSHSRSYKRDDYGSNYWKDSNMRSWLNSTAAEGKVDWLCGNPPKDGYVSGVGAYNEKAGFLNAFSKSEIAAMKTVTQRSLVSHPEYNKGIVDGDANSDLLYYTDISEAVANYDSSYFETTTEKVFLLDVKQANAVWKNLKGYYVAYNNDGMAWPYWLRTPVTDCNHDMRYISSSGQVGRYAPWYSDLGVRPAFYLDSEYFVTTSGSGSQSSPYIGSAPNKQEDDYTISEPAEDANPDWNVSTEQSIQLTLGPWYSNDGKYSNPTIPVYTIQKTRSDTENMVVVVCGEGYTKSQQGKFINDVKRLWQDAMKYEPYRSYADRFNVYALCTASESTFDNGGSTFFDVIVDKYNSPVISNNLHGSQWKNHIFERCIGPEFIEKIHDAHIKKKCDPNTIPSGSEYEPYYYVHDYIAQFAMVVNTKSDFGGAYNNREYGFHYFISPSDSYRASKTFAHEFGHGLLGLGDEYSNGYLLDDKELKSLNLSSVEDPEKIKWRQLLGFRNTYTCRNAYGSKMLVSSYECIMRDTNYQFCEVCRLQGFKRMSQLVKDVDLYVATPEVKEYTGAYSKPSDFTDLETSSYYNYTYNRNDRLLSGNSKSRFNTNMNGKKIELRTVIQNISDKNARQLKFKMWIKHSDGSVATDSSGNPLQTVQTFDIPVWNDKANFWPLGALDHIKSDFNSGLKSCSLIYQIPSDAQLKSGDTVAFQVLDENGNVGGGGSHHHHHHHHHHTCPPCPAPELLGGPSVFLFPPKPKDTLMISRTPEVTCVVVDVSHEDPEVKFNWYVDGVEVHNAKTKPREEQYNSTYRVVSVLTVLHQDWLNGKEYKCKVSNKALPAPIEKTISKAKGQPREPQVYTLPPSRDELTKNQVSLTCLVKGFYPSDIAVEWESNGQPENNYKTTPPVLDSDGSFFLYSKLTVDKSRWQQGNVFSCSVMHEALHNHYTQKSLSLSPGK

SEQ ID NO: 29 - protein, 1015 aa, synthetic construct
ASKPDIKVGDYVKMGVYNNASILWRCVSIDNNGPLMLADKIVDTLAYDAKTNDNSNSKSHSRSYKRDDYGSNYWKDSNMRSWLNSTAAEGKVDWLCGNPPKDGYVSGVGAYNEKAGFLNAFSKSEIAAMKTVTQRSLVSHPEYNKGIVDGDANSDLLYYTDISEAVANYDSSYFETTTEKVFLLDVKQANAVWKNLKGYYVAYNNDGMAWPYWLRTPVTDCNHDMRYISSSGQVGRYAPWYSDLGVRPAFYLDSEYFVTTSGSGSQSSPYIGSAPNKQEDDYTISEPAEDANPDWNVSTEQSIQLTLGPWYSNDGKYSNPTIPVYTIQKTRSDTENMVVVVCGEGYTKSQQGKFINDVKRLWQDAMKYEPYRSYADRFNVYALCTASESTFDNGGSTFFDVIVDKYNSPVISNNLHGSQWKNHIFERCIGPEFIEKIHDAHIKKKCDPNTIPSGSEYEPYYYVHDYIAQFAMVVNTKSDFGGAYNNREYGFHYFISPSDSYRASKTFAHEFGHGLLGLGDEYSNGYLLDDKELKSLNLSSVEDPEKIKWRQLLGFRNTYTCRNAYGSKMLVSSYECIMRDTNYQFCEVCRLQGFKRMSQLVKDVDLYVATPEVKEYTGAYSKPSDFTDLETSSYYNYTYNRNDRLLSGNSKSRFNTNMNGKKIELRTVIQNISDKNARQLKFKMWIKHSDGSVATDSSGNPLQTVQTFDIPVWNDKANFWPLGALDHIKSDFNSGLKSCSLIYQIPSDAQLKSGDTVAFQVLDENGNVLADDNTETQGGGGSHHHHHHHHHHTCPPCPAPELLGGPSVFLFPPKPKDTLMISRTPEVTCVVVDVSHEDPEVKFNWYVDGVEVHNAKTKPREEQYNSTYRVVSVLTVLHQDWLNGKEYKCKVSNKALPAPIEKTISKAKGQPREPQVYTLPPSRDELTKNQVSLTCLVKGFYPSDIAVEWESNGQPENNYKTTPPVLDSDGSFFLYSKLTVDKSRWQQGNVFSCSVMHEALHNHYTQKSLSLSPGK

SEQ ID NO: 30 - protein, 1024 aa, synthetic construct
ASKPDIKVGDYVKMGVYNNASILWRCVSIDNNGPLMLADKIVDTLAYDAKTNDNSNSKSHSRSYKRDDYGSNYWKDSNMRSWLNSTAAEGKVDWLCGNPPKDGYVSGVGAYNEKAGFLNAFSKSEIAAMKTVTQRSLVSHPEYNKGIVDGDANSDLLYYTDISEAVANYDSSYFETTTEKVFLLDVKQANAVWKNLKGYYVAYNNDGMAWPYWLRTPVTDCNHDMRYISSSGQVGRYAPWYSDLGVRPAFYLDSEYFVTTSGSGSQSSPYIGSAPNKQEDDYTISEPAEDANPDWNVSTEQSIQLTLGPWYSNDGKYSNPTIPVYTIQKTRSDTENMVVVVCGEGYTKSQQGKFINDVKRLWQDAMKYEPYRSYADRFNVYALCTASESTFDNGGSTFFDVIVDKYNSPVISNNLHGSQWKNHIFERCIGPEFIEKIHDAHIKKKCDPNTIPSGSEYEPYYYVHDYIAQFAMVVNTKSDFGGAYNNREYGFHYFISPSDSYRASKTFAHEFGHGLLGLGDEYSNGYLLDDKELKSLNLSSVEDPEKIKWRQLLGFRNTYTCRNAYGSKMLVSSYECIMRDTNYQFCEVCRLQGFKRMSQLVKDVDLYVATPEVKEYTGAYSKPSDFTDLETSSYYNYTYNRNDRLLSGNSKSRFNTNMNGKKIELRTVIQNISDKNARQLKFKMWIKHSDGSVATDSSGNPLQTVQTFDIPVWNDKANFWPLGALDHIKSDFNSGLKSCSLIYQIPSDAQLKSGDTVAFQVLDENGNVLADDNTETQRYTTVSIQYGGGGSHHHHHHHHHHTCPPCPAPELLGGPSVFLFPPKPKDTLMISRTPEVTCVVVDVSHEDPEVKFNWYVDGVEVHNAKTKPREEQYNSTYRVVSVLTVLHQDWLNGKEYKCKVSNKALPAPIEKTISKAKGQPREPQVYTLPPSRDELTKNQVSLTCLVKGFYPSDIAVEWESNGQPENNYKTTPPVLDSDGSFFLYSKLTVDKSRWQQGNVFSCSVMHEALHNHYTQKSLSLSPGK

SEQ ID NO: 31 - protein, 1041 aa, synthetic construct
ASKPDIKVGDYVKMGVYNNASILWRCVSIDNNGPLMLADKIVDTLAYDAKTNDNSNSKSHSRSYKRDDYGSNYWKDSNMRSWLNSTAAEGKVDWLCGNPPKDGYVSGVGAYNEKAGFLNAFSKSEIAAMKTVTQRSLVSHPEYNKGIVDGDANSDLLYYTDISEAVANYDSSYFETTTEKVFLLDVKQANAVWKNLKGYYVAYNNDGMAWPYWLRTPVTDCNHDMRYISSSGQVGRYAPWYSDLGVRPAFYLDSEYFVTTSGSGSQSSPYIGSAPNKQEDDYTISEPAEDANPDWNVSTEQSIQLTLGPWYSNDGKYSNPTIPVYTIQKTRSDTENMVVVVCGEGYTKSQQGKFINDVKRLWQDAMKYEPYRSYADRFNVYALCTASESTFDNGGSTFFDVIVDKYNSPVISNNLHGSQWKNHIFERCIGPEFIEKIHDAHIKKKCDPNTIPSGSEYEPYYYVHDYIAQFAMVVNTKSDFGGAYNNREYGFHYFISPSDSYRASKTFAHEFGHGLLGLGDEYSNGYLLDDKELKSLNLSSVEDPEKIKWRQLLGFRNTYTCRNAYGSKMLVSSYECIMRDTNYQFCEVCRLQGFKRMSQLVKDVDLYVATPEVKEYTGAYSKPSDFTDLETSSYYNYTYNRNDRLLSGNSKSRFNTNMNGKKIELRTVIQNISDKNARQLKFKMWIKHSDGSVATDSSGNPLQTVQTFDIPVWNDKANFWPLGALDHIKSDFNSGLKSCSLIYQIPSDAQLKSGDTVAFQVLDENGNVLADDNTETQRYTTVSIQYKFEDGSEIPNTAGGTFTGGGGSHHHHHHHHHHTCPPCPAPELLGGPSVFLFPPKPKDTLMISRTPEVTCVVVDVSHEDPEVKFNWYVDGVEVHNAKTKPREEQYNSTYRVVSVLTVLHQDWLNGKEYKCKVSNKALPAPIEKTISKAKGQPREPQVYTLPPSRDELTKNQVSLTCLVKGFYPSDIAVEWESNGQPENNYKTTPPVLDSDGSFFLYSKLTVDKSRWQQGNVFSCSVMHEALHNHYTQKSLSLSPGK

SEQ ID NO: 32 - protein, 215 aa, synthetic construct
ELLGGPSVFLFPPKPKDTLMISRTPEVTCVVVDVSHEDPEVKFNWYVDGVEVHNAKTKPREEQYNSTYRVVSVLTVLHQDWLNGKEYKCKVSNKALPAPIEKTISKAKGQPREPQVYTLPPSRDELTKNQVSLTCLVKGFYPSDIAVEWESNGQPENNYKTTPPVLDSDGSFFLYSKLTVDKSRWQQGNVFSCSVMHEALHNHYTQKSLSLSPGK

SEQ ID NO: 33 - DNA, 2286 bp, synthetic construct
  source 1..2286: mol_type = other DNA
gcgagcaaaccggacatcaaagtgggcgactacgtgaaaatgggtgtgtataataacgcaagcatcctgtggcgctgtgtgagcatcgacaacaatggcccgctgatgctggccgataaaattgttgacacgctggcgtatgatgctaaaaccaacgacaattcgaacagcaaatctcatagtcgttcctacaaacgcgatgactacggcagcaactattggaaagatagtaatatgcgctcctggctgaactcaaccgcggccgagggtaaagtggattggctgtgcggcaatccgccgaaagacggttacgtcagcggcgtgggtgcatataatgaaaaagctggttttctgaacgcgttctcaaaatcggaaattgcagctatgaaaacggtgacccagcgtagcctggtttctcatccggaatataataaaggcattgttgatggtgacgcgaactcggatctgctgtattacaccgacatcagcgaagcagtggctaactacgatagctcttattttgaaaccacgaccgaaaaagttttcctgctggatgtcaaacaggcgaacgccgtctggaaaaatctgaaaggctattacgtggcttacaacaatgatggtatggcatggccgtattggctgcgtaccccggtgacggattgtaatcatgacatgcgctatattagttcctcaggccaggttggtcgttacgctccgtggtattctgatctgggcgtccgtccggcgttttacctggacagtgaatatttcgtgacgaccagcggctctggtagtcagtcgagcccgtacattggttccgcgccgaacaaacaagaagatgactataccatctcagaaccggcggaagatgccaacccggactggaatgtttcgacggaacagagcattcaactgaccctgggcccgtggtactcgaatgatggtaaatatagcaacccgaccattccggtgtataccatccagaaaacgcgctcggataccgaaaacatggtggttgtcgtgtgcggcgaaggttataccaaatcacagcaaggcaaatttatcaatgatgttaaacgtctgtggcaggacgctatgaaatatgaaccgtaccgtagctatgcggatcgctttaatgtgtatgcactgtgtacggcttccgaatcaaccttcgataacggcggttctacctttttcgatgtgatcgttgacaaatacaactctccggttatcagtaacaatctgcatggcagtcagtggaaaaatcacatttttgaacgctgcatcggtccggaattcattgaaaaaatccatgatgcccacattaagaaaaaatgtgacccgaacaccatcccgtcgggtagcgaatacgaaccgtattactatgtgcatgattatattgcacagtttgctatggttgtcaataccaaatccgacttcggcggtgcatataacaatcgcgaatacggctttcactatttcatctctccgagtgattcctaccgtgcctctaaaacctttgcacatgaattcggccacggtctgctgggcctgggtgatgaatactcgaatggttatctgctggatgacaaagaactgaaaagcctgaacctgtctagtgtggaagatccggaaaaaattaaatggcgtcagctgctgggctttcgcaatacgtacacctgccgtaacgcgtatggttctaaaatgctggtttcctcatacgaatgtatcatgcgcgataccaactatcaattttgcgaagtctgtcgcctgcagggcttcaaacgtatgagccaactggttaaagatgtcgacctgtatgtggccacgccggaagttaaagaatacaccggtgcatatagtaaaccgtccgattttacggacctggaaacctcgagctactacaactacacctacaaccgtaacgatcgcctgctgagtggcaactcaaaatcgcgtttcaatacgaacatgaatggcaagaaaattgaactgcgcaccgttattcagaacatcagcgataaaaacgcccgtcaactgaaattcaaaatgtggatcaaacattcagatggctcggtggcaaccgactctagtggtaacccgctgcagaccgtccaaacgtttgatattccggtgtggaacgacaaagccaatttctggccgctgggcgcactggatcacatcaaatccgactttaattcaggtctgaaaagctgctctctgatttatcagatcccgtctgatgctcaactgaaaagtggcgacaccgtggcgttccaggttctg

SEQ ID NO: 34 - DNA, 2286 bp, synthetic construct; identical to SEQ ID NO: 33
  source 1..2286: mol_type = other DNA

SEQ ID NO: 35 - DNA, 2304 bp, synthetic construct
  source 1..2304: mol_type = other DNA
gcgagcaaaccggacatcaaagtgggcgactacgtgaaaatgggtgtgtataataacgcaagcatcctgtggcgctgtgtgagcatcgacaacaatggcccgctgatgctggccgataaaattgttgacacgctggcgtatgatgctaaaaccaacgacaattcgaacagcaaatctcatagtcgttcctacaaacgcgatgactacggcagcaactattggaaagatagtaatatgcgctcctggctgaactcaaccgcggccgagggtaaagtggattggctgtgcggcaatccgccgaaagacggttacgtcagcggcgtgggtgcatataatgaaaaagctggttttctgaacgcgttctcaaaatcggaaattgcagctatgaaaacggtgacccagcgtagcctggtttctcatccggaatataataaaggcattgttgatggtgacgcgaactcggatctgctgtattacaccgacatcagcgaagcagtggctaactacgatagctcttattttgaaaccacgaccgaaaaagttttcctgctggatgtcaaacaggcgaacgccgtctggaaaaatctgaaaggctattacgtggcttacaacaatgatggtatggcatggccgtattggctgcgtaccccggtgacggattgtaatcatgacatgcgctatattagttcctcaggccaggttggtcgttacgctccgtggtattctgatctgggcgtccgtccggcgttttacctggacagtgaatatttcgtgacgaccagcggctctggtagtcagtcgagcccgtacattggttccgcgccgaacaaacaagaagatgactataccatctcagaaccggcggaagatgccaacccggactggaatgtttcgacggaacagagcattcaactgaccctgggcccgtggtactcgaatgatggtaaatatagcaacccgaccattccggtgtataccatccagaaaacgcgctcggataccgaaaacatggtggttgtcgtgtgcggcgaaggttataccaaatcacagcaaggcaaatttatcaatgatgttaaacgtctgtggcaggacgctatgaaatatgaaccgtaccgtagctatgcggatcgctttaatgtgtatgcactgtgtacggcttccgaatcaaccttcgataacggcggttctacctttttcgatgtgatcgttgacaaatacaactctccggttatcagtaacaatctgcatggcagtcagtggaaaaatcacatttttgaacgctgcatcggtccggaattcattgaaaaaatccatgatgcccacattaagaaaaaatgtgacccgaacaccatcccgtcgggtagcgaatacgaaccgtattactatgtgcatgattatattgcacagtttgctatggttgtcaataccaaatccgacttcggcggtgcatataacaatcgcgaatacggctttcactatttcatctctccgagtgattcctaccgtgcctctaaaacctttgcacatgaattcggccacggtctgctgggcctgggtgatgaatactcgaatggttatctgctggatgacaaagaactgaaaagcctgaacctgtctagtgtggaagatccggaaaaaattaaatggcgtcagctgctgggctttcgcaatacgtacacctgccgtaacgcgtatggttctaaaatgctggtttcctcatacgaatgtatcatgcgcgataccaactatcaattttgcgaagtctgtcgcctgcagggcttcaaacgtatgagccaactggttaaagatgtcgacctgtatgtggccacgccggaagttaaagaatacaccggtgcatatagtaaaccgtccgattttacggacctggaaacctcgagctactacaactacacctacaaccgtaacgatcgcctgctgagtggcaactcaaaatcgcgtttcaatacgaacatgaatggcaagaaaattgaactgcgcaccgttattcagaacatcagcgataaaaacgcccgtcaactgaaattcaaaatgtggatcaaacattcagatggctcggtggcaaccgactctagtggtaacccgctgcagaccgtccaaacgtttgatattccggtgtggaacgacaaagccaatttctggccgctgggcgcactggatcacatcaaatccgactttaattcaggtctgaaaagctgctctctgatttatcagatcccgtctgatgctcaactgaaaagtggcgacaccgtggcgttccaggttctggatgaaaacggtaatgtg

SEQ ID NO: 36 - DNA, 2331 bp, synthetic construct
  source 1..2331: mol_type = other DNA
gcgagcaaaccggacatcaaagtgggcgactacgtgaaaatgggtgtgtataataacgcaagcatcctgtggcgctgtgtgagcatcgacaacaatggcccgctgatgctggccgataaaattgttgacacgctggcgtatgatgctaaaaccaacgacaattcgaacagcaaatctcatagtcgttcctacaaacgcgatgactacggcagcaactattggaaagatagtaatatgcgctcctggctgaactcaaccgcggccgagggtaaagtggattggctgtgcggcaatccgccgaaagacggttacgtcagcggcgtgggtgcatataatgaaaaagctggttttctgaacgcgttctcaaaatcggaaattgcagctatgaaaacggtgacccagcgtagcctggtttctcatccggaatataataaaggcattgttgatggtgacgcgaactcggatctgctgtattacaccgacatcagcgaagcagtggctaactacgatagctcttattttgaaaccacgaccgaaaaagttttcctgctggatgtcaaacaggcgaacgccgtctggaaaaatctgaaaggctattacgtggcttacaacaatgatggtatggcatggccgtattggctgcgtaccccggtgacggattgtaatcatgacatgcgctatattagttcctcaggccaggttggtcgttacgctccgtggtattctgatctgggcgtccgtccggcgttttacctggacagtgaatatttcgtgacgaccagcggctctggtagtcagtcgagcccgtacattggttccgcgccgaacaaacaagaagatgactataccatctcagaaccggcggaagatgccaacccggactggaatgtttcgacggaacagagcattcaactgaccctgggcccgtggtactcgaatgatggtaaatatagcaacccgaccattccggtgtataccatccagaaaacgcgctcggataccgaaaacatggtggttgtcgtgtgcggcgaaggttataccaaatcacagcaaggcaaatttatcaatgatgttaaacgtctgtggcaggacgctatgaaatatgaaccgtaccgtagctatgcggatcgctttaatgtgtatgcactgtgtacggcttccgaatcaaccttcgataacggcggttctacctttttcgatgtgatcgttgacaaatacaactctccggttatcagtaacaatctgcatggcagtcagtggaaaaatcacatttttgaacgctgcatcggtccggaattcattgaaaaaatccatgatgcccacattaagaaaaaatgtgacccgaacaccatcccgtcgggtagcgaatacgaaccgtattactatgtgcatgattatattgcacagtttgctatggttgtcaataccaaatccgacttcggcggtgcatataacaatcgcgaatacggctttcactatttcatctctccgagtgattcctaccgtgcctctaaaacctttgcacatgaattcggccacggtctgctgggcctgggtgatgaatactcgaatggttatctgctggatgacaaagaactgaaaagcctgaacctgtctagtgtggaagatccggaaaaaattaaatggcgtcagctgctgggctttcgcaatacgtacacctgccgtaacgcgtatggttctaaaatgctggtttcctcatacgaatgtatcatgcgcgataccaactatcaattttgcgaagtctgtcgcctgcagggcttcaaacgtatgagccaactggttaaagatgtcgacctgtatgtggccacgccggaagttaaagaatacaccggtgcatatagtaaaccgtccgattttacggacctggaaacctcgagctactacaactacacctacaaccgtaacgatcgcctgctgagtggcaactcaaaatcgcgtttcaatacgaacatgaatggcaagaaaattgaactgcgcaccgttattcagaacatcagcgataaaaacgcccgtcaactgaaattcaaaatgtggatcaaacattcagatggctcggtggcaaccgactctagtggtaacccgctgcagaccgtccaaacgtttgatattccggtgtggaacgacaaagccaatttctggccgctgggcgcactggatcacatcaaatccgactttaattcaggtctgaaaagctgctctctgatttatcagatcccgtctgatgctcaactgaaaagtggcgacaccgtggcgttccaggttctggatgaaaacggtaatgtgctggcggatgacaacacggaaacccag

SEQ ID NO: 37 - DNA, 2358 bp, synthetic construct
  source 1..2358: mol_type = other DNA
gcgagcaaaccggacatcaaagtgggcgactacgtgaaaatgggtgtgtataataacgcaagcatcctgtggcgctgtgtgagcatcgacaacaatggcccgctgatgctggccgataaaattgttgacacgctggcgtatgatgctaaaaccaacgacaattcgaacagcaaatctcatagtcgttcctacaaacgcgatgactacggcagcaactattggaaagatagtaatatgcgctcctggctgaactcaaccgcggccgagggtaaagtggattggctgtgcggcaatccgccgaaagacggttacgtcagcggcgtgggtgcatataatgaaaaagctggttttctgaacgcgttctcaaaatcggaaattgcagctatgaaaacggtgacccagcgtagcctggtttctcatccggaatataataaaggcattgttgatggtgacgcgaactcggatctgctgtattacaccgacatcagcgaagcagtggctaactacgatagctcttattttgaaaccacgaccgaaaaagttttcctgctggatgtcaaacaggcgaacgccgtctggaaaaatctgaaaggctattacgtggcttacaacaatgatggtatggcatggccgtattggctgcgtaccccggtgacggattgtaatcatgacatgcgctatattagttcctcaggccaggttggtcgttacgctccgtggtattctgatctgggcgtccgtccggcgttttacctggacagtgaatatttcgtgacgaccagcggctctggtagtcagtcgagcccgtacattggttccgcgccgaacaaacaagaagatgactataccatctcagaaccggcggaagatgccaacccggactggaatgtttcgacggaacagagcattcaactgaccctgggcccgtggtactcgaatgatggtaaatatagcaacccgaccattccggtgtataccatccagaaaacgcgctcggataccgaaaacatggtggttgtcgtgtgcggcgaaggttataccaaatcacagcaaggcaaatttatcaatgatgttaaacgtctgtggcaggacgctatgaaatatgaaccgtaccgtagctatgcggatcgctttaatgtgtatgcactgtgtacggcttccgaatcaaccttcgataacggcggttctacctttttcgatgtgatcgttgacaaatacaactctccggttatcagtaacaatctgcatggcagtcagtggaaaaatcacatttttgaacgctgcatcggtccggaattcattgaaaaaatccatgatgcccacattaagaaaaaatgtgacccgaacaccatcccgtcgggtagcgaatacgaaccgtattactatgtgcatgattatattgcacagtttgctatggttgtcaataccaaatccgacttcggcggtgcatataacaatcgcgaatacggctttcactatttcatctctccgagtgattcctaccgtgcctctaaaacctttgcacatgaattcggccacggtctgctgggcctgggtgatgaatactcgaatggttatctgctggatgacaaagaactgaaaagcctgaacctgtctagtgtggaagatccggaaaaaattaaatggcgtcagctgctgggctttcgcaatacgtacacctgccgtaacgcgtatggttctaaaatgctggtttcctcatacgaatgtatcatgcgcgataccaactatcaattttgcgaagtctgtcgcctgcagggcttcaaacgtatgagccaactggttaaagatgtcgacctgtatgtggccacgccggaagttaaagaatacaccggtgcatatagtaaaccgtccgattttacggacctggaaacctcgagctactacaactacacctacaaccgtaacgatcgcctgctgagtggcaactcaaaatcgcgtttcaatacgaacatgaatggcaagaaaattgaactgcgcaccgttattcagaacatcagcgataaaaacgcccgtcaactgaaattcaaaatgtggatcaaacattcagatggctcggtggcaaccgactctagtggtaacccgctgcagaccgtccaaacgtttgatattccggtgtggaacgacaaagccaatttctggccgctgggcgcactggatcacatcaaatccgactttaattcaggtctgaaaagctgctctctgatttatcagatcccgtctgatgctcaactgaaaagtggcgacaccgtggcgttccaggttctggatgaaaacggtaatgtgctggcggatgacaacacggaaacccagcgctacacgaccgtttctatccaatac

SEQ ID NO: 38 - DNA, 2409 bp, synthetic construct
  source 1..2409: mol_type = other DNA
gcgagcaaaccggacatcaaagtgggcgactacgtgaaaatgggtgtgtataataacgcaagcatcctgtggcgctgtgtgagcatcgacaacaatggcccgctgatgctggccgataaaattgttgacacgctggcgtatgatgctaaaaccaacgacaattcgaacagcaaatctcatagtcgttcctacaaacgcgatgactacggcagcaactattggaaagatagtaatatgcgctcctggctgaactcaaccgcggccgagggtaaagtggattggctgtgcggcaatccgccgaaagacggttacgtcagcggcgtgggtgcatataatgaaaaagctggttttctgaacgcgttctcaaaatcggaaattgcagctatgaaaacggtgacccagcgtagcctggtttctcatccggaatataataaaggcattgttgatggtgacgcgaactcggatctgctgtattacaccgacatcagcgaagcagtggctaactacgatagctcttattttgaaaccacgaccgaaaaagttttcctgctggatgtcaaacaggcgaacgccgtctggaaaaatctgaaaggctattacgtggcttacaacaatgatggtatggcatggccgtattggctgcgtaccccggtgacggattgtaatcatgacatgcgctatattagttcctcaggccaggttggtcgttacgctccgtggtattctgatctgggcgtccgtccggcgttttacctggacagtgaatatttcgtgacgaccagcggctctggtagtcagtcgagcccgtacattggttccgcgccgaacaaacaagaagatgactataccatctcagaaccggcggaagatgccaacccggactggaatgtttcgacggaacagagcattcaactgaccctgggcccgtggtactcgaatgatggtaaatatagcaacccgaccattccggtgtataccatccagaaaacgcgctcggataccgaaaacatggtggttgtcgtgtgcggcgaaggttataccaaatcacagcaaggcaaatttatcaatgatgttaaacgtctgtggcaggacgctatgaaatatgaaccgtaccgtagctatgcggatcgctttaatgtgtatgcactgtgtacggcttccgaatcaaccttcgataacggcggttctacctttttcgatgtgatcgttgacaaatacaactctccggttatcagtaacaatctgcatggcagtcagtggaaaaatcacatttttgaacgctgcatcggtccggaattcattgaaaaaatccatgatgcccacattaagaaaaaatgtgacccgaacaccatcccgtcgggtagcgaatacgaaccgtattactatgtgcatgattatattgcacagtttgctatggttgtcaataccaaatccgacttcggcggtgcatataacaatcgcgaatacggctttcactatttcatctctccgagtgattcctaccgtgcctctaaaacctttgcacatgaattcggccacggtctgctgggcctgggtgatgaatactcgaatggttatctgctggatgacaaagaactgaaaagcctgaacctgtctagtgtggaagatccggaaaaaattaaatggcgtcagctgctgggctttcgcaatacgtacacctgccgtaacgcgtatggttctaaaatgctggtttcctcatacgaatgtatcatgcgcgataccaactatcaattttgcgaagtctgtcgcctgcagggcttcaaacgtatgagccaactggttaaagatgtcgacctgtatgtggccacgccggaagttaaagaatacaccggtgcatatagtaaaccgtccgattttacggacctggaaacctcgagctactacaactacacctacaaccgtaacgatcgcctgctgagtggcaactcaaaatcgcgtttcaatacgaacatgaatggcaagaaaattgaactgcgcaccgttattcagaacatcagcgataaaaacgcccgtcaactgaaattcaaaatgtggatcaaacattcagatggctcggtggcaaccgactctagtggtaacccgctgcagaccgtccaaacgtttgatattccggtgtggaacgacaaagccaatttctggccgctgggcgcactggatcacatcaaatccgactttaattcaggtctgaaaagctgctctctgatttatcagatcccgtctgatgctcaactgaaaagtggcgacaccgtggcgttccaggttctggatgaaaacggtaatgtgctggcggatgacaacacggaaacccagcgctacacgaccgtttctatccaatacaaattcgaagatggcagtgaaatcccgaatacggcgggcggtaccttcacc

SEQ ID NO: 39 - DNA, 696 bp, synthetic construct
  source 1..696: mol_type = other DNA
gagcccaaatcttgtgacaaaactcacacatgcccaccgtgcccagcacctgaactcctggggggaccgtcagtcttcctcttccccccaaaacccaaggacaccctcatgatctcccggacccctgaggtcacatgcgtggtggtggacgtgagccacgaagaccctgaggtcaagttcaactggtacgtggacggcgtggaggtgcataatgccaagacaaagccgcgggaggagcagtacaacagcacgtaccgggtggtcagcgtcctcaccgtcctgcaccaggactggctgaatggcaaggagtacaagtgcaaggtctccaacaaagccctcccagcccccatcgagaaaaccatctccaaagccaaagggcagccccgagaaccacaggtgtacaccctgcccccatcccgggatgagctgaccaagaaccaggtcagcctgacctgcctggtcaaaggcttctatcccagcgacatcgccgtggagtgggagagcaatgggcagccggagaacaactacaagaccacgcctcccgtgctggactccgacggctccttcttcctctacagcaagctcaccgtggacaagagcaggtggcagcaggggaacgtcttctcatgctccgtgatgcatgaggctctgcacaaccactacacgcagaagagcctctccctgtctccgggtaaa

SEQ ID NO: 40 - DNA, 669 bp, synthetic construct
  source 1..669: mol_type = other DNA
acatgcccaccgtgcccagcacctgaactcctggggggaccgtcagtcttcctcttccccccaaaacccaaggacaccctcatgatctcccggacccctgaggtcacatgcgtggtggtggacgtgagccacgaagaccctgaggtcaagttcaactggtacgtggacggcgtggaggtgcataatgccaagacaaagccgcgggaggagcagtacaacagcacgtaccgggtggtcagcgtcctcaccgtcctgcaccaggactggctgaatggcaaggagtacaagtgcaaggtctccaacaaagccctcccagcccccatcgagaaaaccatctccaaagccaaagggcagccccgagaaccacaggtgtacaccctgcccccatcccgggatgagctgaccaagaaccaggtcagcctgacctgcctggtcaaaggcttctatcccagcgacatcgccgtggagtgggagagcaatgggcagccggagaacaactacaagaccacgcctcccgtgctggactccgacggctccttcttcctctacagcaagctcaccgtggacaagagcaggtggcagcaggggaacgtcttctcatgctccgtgatgcatgaggctctgcacaaccactacacgcagaagagcctctccctgtctccgggtaaa

SEQ ID NO: 41 - DNA, 60 bp, synthetic construct
  source 1..60: mol_type = other DNA
atgtacaggatgcaactcctgtcttgcattgcactaagtcttgcacttgtcacgaattcg

SEQ ID NO: 42 - protein, 1204 aa, synthetic construct
ASKPDIKVGDYVKMGVYNNASILWRCVSIDNNGPLMLADKIVDTLAYDAKTNDNSNSKSHSRSYKRDDYGSNYWKDSNMRSWLNSTAAEGKVDWLCGNPPKDGYVSGVGAYNEKAGFLNAFSKSEIAAMKTVTQRSLVSHPEYNKGIVDGDANSDLLYYTDISEAVANYDSSYFETTTEKVFLLDVKQANAVWKNLKGYYVAYNNDGMAWPYWLRTPVTDCNHDMRYISSSGQVGRYAPWYSDLGVRPAFYLDSEYFVTTSGSGSQSSPYIGSAPNKQEDDYTISEPAEDANPDWNVSTEQSIQLTLGPWYSNDGKYSNPTIPVYTIQKTRSDTENMVVVVCGEGYTKSQQGKFINDVKRLWQDAMKYEPYRSYADRFNVYALCTASESTFDNGGSTFFDVIVDKYNSPVISNNLHGSQWKNHIFERCIGPEFIEKIHDAHIKKKCDPNTIPSGSEYEPYYYVHDYIAQFAMVVNTKSDFGGAYNNREYGFHYFISPSDSYRASKTFAHEFGHGLLGLGDEYSNGYLLDDKELKSLNLSSVEDPEKIKWRQLLGFRNTYTCRNAYGSKMLVSSYECIMRDTNYQFCEVCRLQGFKRMSQLVKDVDLYVATPEVKEYTGAYSKPSDFTDLETSSYYNYTYNRNDRLLSGNSKSRFNTNMNGKKIELRTVIQNISDKNARQLKFKMWIKHSDGSVATDSSGNPLQTVQTFDIPVWNDKANFWPLGALDHIKSDFNSGLKSCSLIYQIPSDAQLKSGDTVAFQVLDENGNVLADDNTETQRYTTVSIQYKFEDGSEIPNTAGGTFTVPYGTKLDLTPAKTLYDYEFIKVDGLNKPIVSDGTVVTYYYKNKNEEHTHNLTLVAAKAATCTTAGNSAYYTCDGCDKWFADATGSVEITDKTSVKIPAPGHTAGTEWKSDDTNHWHECTVAGCGVIIESTKSAHTAGEWIVDTPATATTAGTKHKECTVCHRVLETQPIPSTGTELKIIAGDNQIYNKASGSDVTITCNGDFAKFTGIKVDGSVVDSSNYTAVSGSTVLTLKASYLGTLTDGSHTITFVYTDGEANANLTVRTAGSGHIHDYGTEWKSNADNHWHECNCGDKKDEAAHSFKWVVDKEATATKKGSKHEECKICGYKRSAVEIPATGTSTAPTDTTKPNDTTKPGNTNGSEKSPQTGDNSNIFLWFALLFVSAAGVTGITAYNKKKKEHAE

SEQ ID NO: 43 - protein, 506 aa, synthetic construct
EYFVTTSGSGSQSSPYIGSAPNKQEDDYTISEPAEDANPDWNVSTEQSIQLTLGPWYSNDGKYSNPTIPVYTIQKTRSDTENMVVVVCGEGYTKSQQGKFINDVKRLWQDAMKYEPYRSYADRFNVYALCTASESTFDNGGSTFFDVIVDKYNSPVISNNLHGSQWKNHIFERCIGPEFIEKIHDAHIKKKCDPNTIPSGSEYEPYYYVHDYIAQFAMVVNTKSDFGGAYNNREYGFHYFISPSDSYRASKTFAHEFGHGLLGLGDEYSNGYLLDDKELKSLNLSSVEDPEKIKWRQLLGFRNTYTCRNAYGSKMLVSSYECIMRDTNYQFCEVCRLQGFKRMSQLVKDVDLYVATPEVKEYTGAYSKPSDFTDLETSSYYNYTYNRNDRLLSGNSKSRFNTNMNGKKIELRTVIQNISDKNARQLKFKMWIKHSDGSVATDSSGNPLQTVQTFDIPVWNDKANFWPLGALDHIKSDFNSGLKSCSLIYQIPSDAQLKSGDTVAFQ

SEQ ID NO: 44 - protein, 507 aa, synthetic construct
EYFVTTSGSGSQSSPYIGSAPNKQEDDYTISEPAEDANPDWNVSTEQSIQLTLGPWYSNDGKYSNPTIPVYTIQKTRSDTENMVVVVCGEGYTKSQQGKFINDVKRLWQDAMKYEPYRSYADRFNVYALCTASESTFDNGGSTFFDVIVDKYNSPVISNNLHGSQWKNHIFERCIGPEFIEKIHDAHIKKKCDPNTIPSGSEYEPYYYVHDYIAQFAMVVNTKSDFGGAYNNREYGFHYFISPSDSYRASKTFAHEFGHGLLGLGDEYSNGYLLDDKELKSLNLSSVEDPEKIKWRQLLGFRNTYTCRNAYGSKMLVSSYECIMRDTNYQFCEVCRLQGFKRMSQLVKDVDLYVATPEVKEYTGAYSKPSDFTDLETSSYYNYTYNRNDRLLSGNSKSRFNTNMNGKKIELRTVIQNISDKNARQLKFKMWIKHSDGSVATDSSGNPLQTVQTFDIPVWNDKANFWPLGALDHIKSDFNSGLKSCSLIYQIPSDAQLKSGDTVAFQV

SEQ ID NO: 45 - protein, 508 aa, synthetic construct
EYFVTTSGSGSQSSPYIGSAPNKQEDDYTISEPAEDANPDWNVSTEQSIQLTLGPWYSNDGKYSNPTIPVYTIQKTRSDTENMVVVVCGEGYTKSQQGKFINDVKRLWQDAMKYEPYRSYADRFNVYALCTASESTFDNGGSTFFDVIVDKYNSPVISNNLHGSQWKNHIFERCIGPEFIEKIHDAHIKKKCDPNTIPSGSEYEPYYYVHDYIAQFAMVVNTKSDFGGAYNNREYGFHYFISPSDSYRASKTFAHEFGHGLLGLGDEYSNGYLLDDKELKSLNLSSVEDPEKIKWRQLLGFRNTYTCRNAYGSKMLVSSYECIMRDTNYQFCEVCRLQGFKRMSQLVKDVDLYVATPEVKEYTGAYSKPSDFTDLETSSYYNYTYNRNDRLLSGNSKSRFNTNMNGKKIELRTVIQNISDKNARQLKFKMWIKHSDGSVATDSSGNPLQTVQTFDIPVWNDKANFWPLGALDHIKSDFNSGLKSCSLIYQIPSDAQLKSGDTVAFQVL

SEQ ID NO: 46 - protein, 532 aa, synthetic construct
EYFVTTSGSGSQSSPYIGSAPNKQEDDYTISEPAEDANPDWNVSTEQSIQLTLGPWYSNDGKYSNPTIPVYTIQKTRSDTENMVVVVCGEGYTKSQQGKFINDVKRLWQDAMKYEPYRSYADRFNVYALCTASESTFDNGGSTFFDVIVDKYNSPVISNNLHGSQWKNHIFERCIGPEFIEKIHDAHIKKKCDPNTIPSGSEYEPYYYVHDYIAQFAMVVNTKSDFGGAYNNREYGFHYFISPSDSYRASKTFAHEFGHGLLGLGDEYSNGYLLDDKELKSLNLSSVEDPEKIKWRQLLGFRNTYTCRNAYGSKMLVSSYECIMRDTNYQFCEVCRLQGFKRMSQLVKDVDLYVATPEVKEYTGAYSKPSDFTDLETSSYYNYTYNRNDRLLSGNSKSRFNTNMNGKKIELRTVIQNISDKNARQLKFKMWIKHSDGSVATDSSGNPLQTVQTFDIPVWNDKANFWPLGALDHIKSDFNSGLKSCSLIYQIPSDAQLKSGDTVAFQVLDENGNVLADDNTETQRYTTVSIQY

SEQ ID NO: 47 - protein, 461 aa, synthetic construct
EQSIQLTLGPWYSNDGKYSNPTIPVYTIQKTRSDTENMVVVVCGEGYTKSQQGKFINDVKRLWQDAMKYEPYRSYADRFNVYALCTASESTFDNGGSTFFDVIVDKYNSPVISNNLHGSQWKNHIFERCIGPEFIEKIHDAHIKKKCDPNTIPSGSEYEPYYYVHDYIAQFAMVVNTKSDFGGAYNNREYGFHYFISPSDSYRASKTFAHEFGHGLLGLGDEYSNGYLLDDKELKSLNLSSVEDPEKIKWRQLLGFRNTYTCRNAYGSKMLVSSYECIMRDTNYQFCEVCRLQGFKRMSQLVKDVDLYVATPEVKEYTGAYSKPSDFTDLETSSYYNYTYNRNDRLLSGNSKSRFNTNMNGKKIELRTVIQNISDKNARQLKFKMWIKHSDGSVATDSSGNPLQTVQTFDIPVWNDKANFWPLGALDHIKSDFNSGLKSCSLIYQIPSDAQLKSGDTVAFQ

SEQ ID NO: 48 - protein, 462 aa, synthetic construct
EQSIQLTLGPWYSNDGKYSNPTIPVYTIQKTRSDTENMVVVVCGEGYTKSQQGKFINDVKRLWQDAMKYEPYRSYADRFNVYALCTASESTFDNGGSTFFDVIVDKYNSPVISNNLHGSQWKNHIFERCIGPEFIEKIHDAHIKKKCDPNTIPSGSEYEPYYYVHDYIAQFAMVVNTKSDFGGAYNNREYGFHYFISPSDSYRASKTFAHEFGHGLLGLGDEYSNGYLLDDKELKSLNLSSVEDPEKIKWRQLLGFRNTYTCRNAYGSKMLVSSYECIMRDTNYQFCEVCRLQGFKRMSQLVKDVDLYVATPEVKEYTGAYSKPSDFTDLETSSYYNYTYNRNDRLLSGNSKSRFNTNMNGKKIELRTVIQNISDKNARQLKFKMWIKHSDGSVATDSSGNPLQTVQTFDIPVWNDKANFWPLGALDHIKSDFNSGLKSCSLIYQIPSDAQLKSGDTVAFQV

SEQ ID NO: 49 - protein, 463 aa, synthetic construct
EQSIQLTLGPWYSNDGKYSNPTIPVYTIQKTRSDTENMVVVVCGEGYTKSQQGKFINDVKRLWQDAMKYEPYRSYADRFNVYALCTASESTFDNGGSTFFDVIVDKYNSPVISNNLHGSQWKNHIFERCIGPEFIEKIHDAHIKKKCDPNTIPSGSEYEPYYYVHDYIAQFAMVVNTKSDFGGAYNNREYGFHYFISPSDSYRASKTFAHEFGHGLLGLGDEYSNGYLLDDKELKSLNLSSVEDPEKIKWRQLLGFRNTYTCRNAYGSKMLVSSYECIMRDTNYQFCEVCRLQGFKRMSQLVKDVDLYVATPEVKEYTGAYSKPSDFTDLETSSYYNYTYNRNDRLLSGNSKSRFNTNMNGKKIELRTVIQNISDKNARQLKFKMWIKHSDGSVATDSSGNPLQTVQTFDIPVWNDKANFWPLGALDHIKSDFNSGLKSCSLIYQIPSDAQLKSGDTVAFQVL

SEQ ID NO: 50 - protein, 456 aa, synthetic construct
LTLGPWYSNDGKYSNPTIPVYTIQKTRSDTENMVVVVCGEGYTKSQQGKFINDVKRLWQDAMKYEPYRSYADRFNVYALCTASESTFDNGGSTFFDVIVDKYNSPVISNNLHGSQWKNHIFERCIGPEFIEKIHDAHIKKKCDPNTIPSGSEYEPYYYVHDYIAQFAMVVNTKSDFGGAYNNREYGFHYFISPSDSYRASKTFAHEFGHGLLGLGDEYSNGYLLDDKELKSLNLSSVEDPEKIKWRQLLGFRNTYTCRNAYGSKMLVSSYECIMRDTNYQFCEVCRLQGFKRMSQLVKDVDLYVATPEVKEYTGAYSKPSDFTDLETSSYYNYTYNRNDRLLSGNSKSRFNTNMNGKKIELRTVIQNISDKNARQLKFKMWIKHSDGSVATDSSGNPLQTVQTFDIPVWNDKANFWPLGALDHIKSDFNSGLKSCSLIYQIPSDAQLKSGDTVAFQ

SEQ ID NO: 51 - protein, 457 aa, synthetic construct
LTLGPWYSNDGKYSNPTIPVYTIQKTRSDTENMVVVVCGEGYTKSQQGKFINDVKRLWQDAMKYEPYRSYADRFNVYALCTASESTFDNGGSTFFDVIVDKYNSPVISNNLHGSQWKNHIFERCIGPEFIEKIHDAHIKKKCDPNTIPSGSEYEPYYYVHDYIAQFAMVVNTKSDFGGAYNNREYGFHYFISPSDSYRASKTFAHEFGHGLLGLGDEYSNGYLLDDKELKSLNLSSVEDPEKIKWRQLLGFRNTYTCRNAYGSKMLVSSYECIMRDTNYQFCEVCRLQGFKRMSQLVKDVDLYVATPEVKEYTGAYSKPSDFTDLETSSYYNYTYNRNDRLLSGNSKSRFNTNMNGKKIELRTVIQNISDKNARQLKFKMWIKHSDGSVATDSSGNPLQTVQTFDIPVWNDKANFWPLGALDHIKSDFNSGLKSCSLIYQIPSDAQLKSGDTVAFQV

SEQ ID NO: 52 - protein, 458 aa, synthetic construct
LTLGPWYSNDGKYSNPTIPVYTIQKTRSDTENMVVVVCGEGYTKSQQGKFINDVKRLWQDAMKYEPYRSYADRFNVYALCTASESTFDNGGSTFFDVIVDKYNSPVISNNLHGSQWKNHIFERCIGPEFIEKIHDAHIKKKCDPNTIPSGSEYEPYYYVHDYIAQFAMVVNTKSDFGGAYNNREYGFHYFISPSDSYRASKTFAHEFGHGLLGLGDEYSNGYLLDDKELKSLNLSSVEDPEKIKWRQLLGFRNTYTCRNAYGSKMLVSSYECIMRDTNYQFCEVCRLQGFKRMSQLVKDVDLYVATPEVKEYTGAYSKPSDFTDLETSSYYNYTYNRNDRLLSGNSKSRFNTNMNGKKIELRTVIQNISDKNARQLKFKMWIKHSDGSVATDSSGNPLQTVQTFDIPVWNDKANFWPLGALDHIKSDFNSGLKSCSLIYQIPSDAQLKSGDTVAFQVL

SEQ ID NO: 53 - protein, 1173 aa, synthetic construct
ASKPDIKVGDYVKMGVYNNASILWRCVSIDNNGPLMLADKIVDTLAYDAKTNDNSNSKSHSRSYKRDDYGSNYWKDSNMRSWLNSTAAEGKVDWLCGNPPKDGYVSGVGAYNEKAGFLNAFSKSEIAAMKTVTQRSLVSHPEYNKGIVDGDANSDLLYYTDISEAVANYDSSYFETTTEKVFLLDVKQANAVWKNLKGYYVAYNNDGMAWPYWLRTPVTDCNHDMRYISSSGQVGRYAPWYSDLGVRPAFYLDSEYFVTTSGSGSQSSPYIGSAPNKQEDDYTISEPAEDANPDWNVSTEQSIQLTLGPWYSNDGKYSNPTIPVYTIQKTRSDTENMVVVVCGEGYTKSQQGKFINDVKRLWQDAMKYEPYRSYADRFNVYALCTASESTFDNGGSTFFDVIVDKYNSPVISNNLHGSQWKNHIFERCIGPEFIEKIHDAHIKKKCDPNTIPSGSEYEPYYYVHDYIAQFAMVVNTKSDFGGAYNNREYGFHYFISPSDSYRASKTFAHEFGHGLLGLGDEYSNGYLLDDKELKSLNLSSVEDPEKIKWRQLLGFRNTYTCRNAYGSKMLVSSYECIMRDTNYQFCEVCRLQGFKRMSQLVKDVDLYVATPEVKEYTGAYSKPSDFTDLETSSYYNYTYNRNDRLLSGNSKSRFNTNMNGKKIELRTVIQNISDKNARQLKFKMWIKHSDGSVATDSSGNPLQTVQTFDIPVWNDKANFWPLGALDHIKSDFNSGLKSCSLIYQIPSDAQLKSGDTVAFQVLDENGNVLADDNTETQRYTTVSIQYKFEDGSEIPNTAGGTFTVPYGTKLDLTGAKTLYDYEFIKVDGLNKPIVSDGTVVTYYYKNKNEEHTHNLTLVAAKAATCTTAGNSAYYTCDGCDKWFADATGSVEITDKTSVKIPAPGHTAGTEWKSDDTNHWHECTVAGCGVIIESTKSAHTAGEWIVDTPATATTAGTKHKECTVCHRVLETQPIPSTGTELKIIAGDNQIYNKASGSDVTITCNGDFAKFTGIKVDGSVVDSSNYTAVSGSTVLTLKASYLGTLTDGSHTITFVYTDGEANANLTVRTAGSGHIHDYGTEWKSNADNHWHECNCGDKKDEAAHSFKWVVDKEATATKKGSKHEECKICGYKRSAVEIPATGTSTAPTDTTKPNDTTKPGNTNGSEKSPQTGDNS

SEQ ID NO: 54 - protein, 1173 aa, synthetic construct
ASKPDIKVGDYVKMGVYNNASILWRCVSIDNNGPLMLADKIVDTLAYDAKTNDNSNSKSHSRSYKRDDYGSNYWKDSNMRSWLNSTAAEGKVDWLCGNPPKDGYVSGVGAYNEKAGFLNAFSKSEIAAMKTVTQRSLVSHPEYNKGIVDGDANSDLLYYTDISEAVANYDSSYFETTTEKVFLLDVKQANAVWKNLKGYYVAYNNDGMAWPYWLRTPVTDCNHDMRYISSSGQVGRYAPWYSDLGVRPAFYLDSEYFVTTSGSGSQSSPYIGSAPNKQEDDYTISEPAEDANPDWNVSTEQSIQLTLGPWYSNDGKYSNPTIPVYTIQKTRSDTENMVVVVCGEGYTKSQQGKFINDVKRLWQDAMKYEPYRSYADRFNVYALCTASESTFDNGGSTFFDVIVDKYNSPVISNNLHGSQWKNHIFERCIGPEFIEKIHDAHIKKKCDPNTIPSGSEYEPYYYVHDYIAQFAMVVNTKSDFGGAYNNREYGFHYFISPSDSYRASKTFAHEFGHGLLGLGDEYSNGYLLDDKELKSLNLSSVEDPEKIKWRQLLGFRNTYTCRNAYGSKMLVSSYECIMRDTNYQFCEVCRLQGFKRMSQLVKDVDLYVATPEVKEYTGAYSKPSDFTDLETSSYYNYTYNRNDRLLSGNSKSRFNTNMNGKKIELRTVIQNISDKNARQLKFKMWIKHSDGSVATDSSGNPLQTVQTFDIPVWNDKANFWPLGALDHIKSDFNSGLKSCSLIYQIPSDAQLKSGDTVAFQVLDENGNVLADDNTETQRYTTVSIQYKFEDGSEIPNTAGGTFTVPYGTKLDLTPAKTLYDYEFIKVDGLNKGIVSDGTVVTYYYKNKNEEHTHNLTLVAAKAATCTTAGNSAYYTCDGCDKWFADATGSVEITDKTSVKIPAPGHTAGTEWKSDDTNHWHECTVAGCGVIIESTKSAHTAGEWIVDTPATATTAGTKHKECTVCHRVLETQPIPSTGTELKIIAGDNQIYNKASGSDVTITCNGDFAKFTGIKVDGSVVDSSNYTAVSGSTVLTLKASYLGTLTDGSHTITFVYTDGEANANLTVRTAGSGHIHDYGTEWKSNADNHWHECNCGDKKDEAAHSFKWVVDKEATATKKGSKHEECKICGYKRSAVEIPATGTSTAPTDTTKPNDTTKPGNTNGSEKSPQTGDNS

SEQ ID NO: 55 - protein, 1173 aa, synthetic construct
ASKPDIKVGDYVKMGVYNNASILWRCVSIDNNGPLMLADKIVDTLAYDAKTNDNSNSKSHSRSYKRDDYGSNYWKDSNMRSWLNSTAAEGKVDWLCGNPPKDGYVSGVGAYNEKAGFLNAFSKSEIAAMKTVTQRSLVSHPEYNKGIVDGDANSDLLYYTDISEAVANYDSSYFETTTEKVFLLDVKQANAVWKNLKGYYVAYNNDGMAWPYWLRTPVTDCNHDMRYISSSGQVGRYAPWYSDLGVRPAFYLDSEYFVTTSGSGSQSSPYIGSAPNKQEDDYTISEPAEDANPDWNVSTEQSIQLTLGPWYSNDGKYSNPTIPVYTIQKTRSDTENMVVVVCGEGYTKSQQGKFINDVKRLWQDAMKYEPYRSYADRFNVYALCTASESTFDNGGSTFFDVIVDKYNSPVISNNLHGSQWKNHIFERCIGPEFIEKIHDAHIKKKCDPNTIPSGSEYEPYYYVHDYIAQFAMVVNTKSDFGGAYNNREYGFHYFISPSDSYRASKTFAHEFGHGLLGLGDEYSNGYLLDDKELKSLNLSSVEDPEKIKWRQLLGFRNTYTCRNAYGSKMLVSSYECIMRDTNYQFCEVCRLQGFKRMSQLVKDVDLYVATPEVKEYTGAYSKPSDFTDLETSSYYNYTYNRNDRLLSGNSKSRFNTNMNGKKIELRTVIQNISDKNARQLKFKMWIKHSDGSVATDSSGNPLQTVQTFDIPVWNDKANFWPLGALDHIKSDFNSGLKSCSLIYQIPSDAQLKSGDTVAFQVLDENGNVLADDNTETQRYTTVSIQYKFEDGSEIPNTAGGTFTVPYGTKLDLTPAKTLYDYEFIKVDGLNKPIVSDGTVVTYYYKNKNEEHTHNLTLVAAKAATCTTAGNSAYYTCDGCDKWFADATGSVEITDKTSVKIGAGGHTAGTEWKSDDTNHWHECTVAGCGVIIESTKSAHTAGEWIVDTPATATTAGTKHKECTVCHRVLETQPIPSTGTELKIIAGDNQIYNKASGSDVTITCNGDFAKFTGIKVDGSVVDSSNYTAVSGSTVLTLKASYLGTLTDGSHTITFVYTDGEANANLTVRTAGSGHIHDYGTEWKSNADNHWHECNCGDKKDEAAHSFKWVVDKEATATKKGSKHEECKICGYKRSAVEIPATGTSTAPTDTTKPNDTTKPGNTNGSEKSPQTGDNS

SEQ ID NO: 56 - protein, 1173 aa, synthetic construct
ASKPDIKVGDYVKMGVYNNASILWRCVSIDNNGPLMLADKIVDTLAYDAKTNDNSNSKSHSRSYKRDDYGSNYWKDSNMRSWLNSTAAEGKVDWLCGNPPKDGYVSGVGAYNEKAGFLNAFSKSEIAAMKTVTQRSLVSHPEYNKGIVDGDANSDLLYYTDISEAVANYDSSYFETTTEKVFLLDVKQANAVWKNLKGYYVAYNNDGMAWPYWLRTPVTDCNHDMRYISSSGQVGRYAPWYSDLGVRPAFYLDSEYFVTTSGSGSQSSPYIGSAPNKQEDDYTISEPAEDANPDWNVSTEQSIQLTLGPWYSNDGKYSNPTIPVYTIQKTRSDTENMVVVVCGEGYTKSQQGKFINDVKRLWQDAMKYEPYRSYADRFNVYALCTASESTFDNGGSTFFDVIVDKYNSPVISNNLHGSQWKNHIFERCIGPEFIEKIHDAHIKKKCDPNTIPSGSEYEPYYYVHDYIAQFAMVVNTKSDFGGAYNNREYGFHYFISPSDSYRASKTFAHEFGHGLLGLGDEYSNGYLLDDKELKSLNLSSVEDPEKIKWRQLLGFRNTYTCRNAYGSKMLVSSYECIMRDTNYQFCEVCRLQGFKRMSQLVKDVDLYVATPEVKEYTGAYSKPSDFTDLETSSYYNYTYNRNDRLLSGNSKSRFNTNMNGKKIELRTVIQNISDKNARQLKFKMWIKHSDGSVATDSSGNPLQTVQTFDIPVWNDKANFWPLGALDHIKSDFNSGLKSCSLIYQIPSDAQLKSGDTVAFQVLDENGNVLADDNTETQRYTTVSIQYKFEDGSEIPNTAGGTFTVPYGTKLDLTPAKTLYDYEFIKVDGLNKPIVSDGTVVTYYYKNKNEEHTHNLTLVAAKAATCTTAGNSAYYTCDGCDKWFADATGSVEITDKTSVKIPAPGHTAGTEWKSDDTNHWHECTVAGCGVIIESTKSAHTAGEWIVDTGATATTAGTKHKECTVCHRVLETQPIPSTGTELKIIAGDNQIYNKASGSDVTITCNGDFAKFTGIKVDGSVVDSSNYTAVSGSTVLTLKASYLGTLTDGSHTITFVYTDGEANANLTVRTAGSGHIHDYGTEWKSNADNHWHECNCGDKKDEAAHSFKWVVDKEATATKKGSKHEECKICGYKRSAVEIPATGTSTAPTDTTKPNDTTKPGNTNGSEKSPQTGDNS

SEQ ID NO: 57 - protein, 1173 aa, synthetic construct
ASKPDIKVGDYVKMGVYNNASILWRCVSIDNNGPLMLADKIVDTLAYDAKTNDNSNSKSHSRSYKRDDYGSNYWKDSNMRSWLNSTAAEGKVDWLCGNPPKDGYVSGVGAYNEKAGFLNAFSKSEIAAMKTVTQRSLVSHPEYNKGIVDGDANSDLLYYTDISEAVANYDSSYFETTTEKVFLLDVKQANAVWKNLKGYYVAYNNDGMAWPYWLRTPVTDCNHDMRYISSSGQVGRYAPWYSDLGVRPAFYLDSEYFVTTSGSGSQSSPYIGSAPNKQEDDYTISEPAEDANPDWNVSTEQSIQLTLGPWYSNDGKYSNPTIPVYTIQKTRSDTENMVVVVCGEGYTKSQQGKFINDVKRLWQDAMKYEPYRSYADRFNVYALCTASESTFDNGGSTFFDVIVDKYNSPVISNNLHGSQWKNHIFERCIGPEFIEKIHDAHIKKKCDPNTIPSGSEYEPYYYVHDYIAQFAMVVNTKSDFGGAYNNREYGFHYFISPSDSYRASKTFAHEFGHGLLGLGDEYSNGYLLDDKELKSLNLSSVEDPEKIKWRQLLGFRNTYTCRNAYGSKMLVSSYECIMRDTNYQFCEVCRLQGFKRMSQLVKDVDLYVATPEVKEYTGAYSKPSDFTDLETSSYYNYTYNRNDRLLSGNSKSRFNTNMNGKKIELRTVIQNISDKNARQLKFKMWIKHSDGSVATDSSGNPLQTVQTFDIPVWNDKANFWPLGALDHIKSDFNSGLKSCSLIYQIPSDAQLKSGDTVAFQVLDENGNVLADDNTETQRYTTVSIQYKFEDGSEIPNTAGGTFTVPYGTKLDLTPAKTLYDYEFIKVDGLNKPIVSDGTVVTYYYKNKNEEHTHNLTLVAAKAATCTTAGNSAYYTCDGCDKWFADATGSVEITDKTSVKIPAPGHTAGTEWKSDDTNHWHECTVAGCGVIIESTKSAHTAGEWIVDTPATATTAGTKHKECTVCHRVLETQGIGSTGTELKIIAGDNQIYNKASGSDVTITCNGDFAKFTGIKVDGSVVDSSNYTAVSGSTVLTLKASYLGTLTDGSHTITFVYTDGEANANLTVRTAGSGHIHDYGTEWKSNADNHWHECNCGDKKDEAAHSFKWVVDKEATATKKGSKHEECKICGYKRSAVEIPATGTSTAPTDTTKPNDTTKPGNTNGSEKSPQTGDNS

SEQ ID NO: 58 - protein, 18 aa, synthetic construct
EEKKKEKEKEEQEERETK

SEQ ID NO: 59 - protein, 10 aa, synthetic construct
HHHHHHHHHH

SEQ ID NO: 60 - protein, 585 aa, synthetic construct [sequence omitted]

SEQ ID NO: 61 - protein, 916 aa, Hominisplanchenecus faecis
MTKKITAIFLALCMAISVLPITIQAASKPDIKVGDYVKMGAYNNASILWRCVSIDNNGPLMLADKIVDTLAYDAKTNDNSNSKSHSRSYKRDDYGSNYWKDSNMRSWLNSTAAEGKVDWLCGNPPKDGYVSGVGAYNEKAGFLNAFSKSEIAAMKTVTQRSLVSHPEYNKGIVDGDANSDLLYYTDISEAVANYDSSYFETTTEKVFLLDVKQANAVWKNLKGYYVAYNNDGMAWPYWLRTPVTDCNHDMRYISSSGQVGRYAPWYSDLGVRPAFYLDSEYFVTTSGSGSQSSPYIGSAPNKQEDDYTISEPAEDANPDWNVSTEQSIQLTLGPWYSNDGKYSNPTIPVYTIQKTRSDTENMVVVVCGEGYTKSQQGKFINDVKRLWQDAMKYEPYRSYADRFNVYALCTASESTFDNGGSTFFDVIVDKYNSPVISNNLHGSQWKNHIFERCIGPEFIEKIHDAHIKKKCDPNTIPSGSEYEPYYYVHDYIAQFAMVVNTKSDFGGAYNNREYGFHYFISPSDSYRASKTFAHEFGHGLLGLGDEYSNGYLLDDKELKSLNLSSVEDPEKIKWRQLLGFRNTYTCRNAYGSKMLVSSYECIMRDTNYQFCEVCRLQGFKRMSQLVKDVDLYVATPEVKEYTGAYSKPSDFTDLETSSYYNYTYNRNDRLLSGNSKSRFNTNMNGKKIELRTVIQNISDKNARQLKFKMWIKHSDGSVATDSSGNPLQTVQTFDIPVWNDKANFWPLGALDHIKSDFNSGLKSCSLIYQIPSDAQLKSGDTVAFQVLDENGNVLADDNTETQRYTTVSIQYKFEDGSEIPNTAGGTFTVPYGTKLDLTPAKTLYDYEFIKVDGLNKPIVSDGTVVTYYYKNKNEEHTHNLTLVAAKAATCITAGNSAYYTCDGCDKWFADATGSVE

SEQ ID NO: 62 - protein, 1214 aa, Roseburia intestinalis
MTKKITAIFLALCMAISVLPMTIQAASKPDIKVGDYVKMGAYNNASILWRCVSIDNNGPLMLADKIVDTLAYDAKTNDNSNSKSHSRSYKRDDYGSNYWKDSNMRSWLNSTAAEGKVDWLCGNPPKDGYVSGVGAYNEKAGFLNAFSKSEIAAMKTVTQRSLVSHPEYNKGIVDGDANSDLLYYTDISEAVANYDSSYFETTTEKVFLLDVKQANAVWKNLKGYYVAYNNDGMAWPYWLRTPVTDCNHDMRYISSSGQVGRYAPWYSDLGVRPAFYLDSEYFVTTSGSGSQSSPYIGSAPNKQEDDYTISEPAEDANPDWNVSTEQSIQLTLGPWYSNDGKYSNPTIPVYTIQKTRSDTENMVVVVCGEGYTKSQQGKFINDVKRLWQDAMKYEPYRSYADRFNVYALCTASESTFDNGGSTFFDVIVDKHNSPVISNNLHGSQWKNHIFERCIGPEFIEKIHDAHIKKKCDPNTIPSGSEYEPYYYVHDYIAQFAMVVNTKSDFGGAYNNREYGFHYFISPSDSYRASKTFAHEFGHGLLGLGDEYSDGYLLDDKELKSLNLSSVEDPEKIKWRQLLGFRNTYTCRNAYGSKMLVSSYECIMRDTNYQFCEVCRLQGFKRMSQLVKDVDLYVATPEVKEYTGAYSKPSDFTDLETSSYYNYTYNRNDRLLSGNSKSRFNTNMNGKKIELRTVIQNISDKNARQLKFKMWIKHSDGSVATDSSGNPLQTVQTFDIPVWNDKANFWPLGALDHIKSDFNSGLKSCSLIYQIPSDAQLKSGDTVAFQVLDENGNVLADDNTETQRYTTVSIQYKFEDGSEIPNTAGGTFTVPYGTKLDLTPAKTLYDYEFIKVDGLNKPIVSDGTVVTYYYKNKNEEHTHNLTLVAAKAATCTTAGNSAYYTCDGCDKWFADATGSVEITDKTSVKIPAPGHTAGTEWKSDDTNHWHECSRCHDKKDEAAHDYGSDNVCDTCGYYKTVPHTHNLTLVAAKAATCTESGKEAYYKCEGCGKFYEDVLGTKEITDLASWGNIAKIAHTTKQTVTKASSIKLKATSLTYNGKVRTPKVIVKDRTGKTLVKNTDYTVSYAKGRKYVGKYAVKITFKGKYSGTKTLYFTIKPKATSISSLKAGSKKFTVKWKKQATQTTGYQVQYSASSKFSKAKTVTVGKNTTVSKKISKLSGKKKYYVRVRTYKTVKINGKSIRIYSGWSKAKTVTTKK

SEQ ID NO: 63 - protein, 1174 aa, Eubacterium ventriosum
MTKKITAIFLALCMAISVLPMTIQAASKPDIKVGDYVKMGAYNNASILWRCVSIDNNGPLMLADKIVDTLAYDAKTNDNSNSKSHSRSYKRDDYGSNYWKDSNMRSWLNSTAAEGKVDWLCGNPPKDGYVSGVGAYNEKAGFLNAFSKSEIAAMKTVTQRSLVSHPEYNKGIVDGDANSDLLYYTDISEAVANYDSSYFETTTEKVFLLDVKQANAVWKNLKGYYVAYNNDGMAWPYWLRTPVTDCNHDMRYISSSGQVGRYAPWYSDLGVRPAFYLDSEYFVTTSGSGSQSSPYIGSAPNKQEDDYTISEPAEDANPDWNVSTEQSIQLTLGPWYSNDGKYSNPTIPVYTIQKTRSDTENMVVVVCGEGYTKSQQGKFINDVKRLWQDAMKYEPYRSYADRFNVYALCTASESTFDNGGSTFFDVIVDKYNSPVISNNLHGSQWKNHIFERCIGPEFIEKIHDAHIKKKCDPNTIPSGSEYEPYYYVHDYIAQFAMVVNTKSDFGGAYNNREYGFHYFISPSDSYRASKTFAHEFGHGLLGLGDEYSNGYLLDDKELKSLNLSSVEDPEKIKWRQFLGFRNTYTCRNAYGSKMLVSSYECIMRDTNYQFCEVCRLQGFKRMSQLVKDVDLYVATPEVKEYTGAYSKPSDFTDLETSSYYNYTYNRNDRLLSGNSKSRFNTNMNGKKIELRTVIQNISDKNARQLKFKMWIKHSDGSVATDSSGNPLQTVQTFDIPVWNDKANFWPLGALDHIKSDFNSGLKSCSLIYQIPSDAQLKSGDTVAFQVLDENGNVLADDNTETQRYTTVSIQYKFEDGSEIPNTAGGTFTVPYGTKLDLTPAKTLYDYEFIKVDGLNKPIVSDGTVVTYYYKNKNEEHTHNLTLVAAKAATCTTAGNSAYYTCDGCDKWFADATGSIEITDKTSVKIPAPGHTAGTEWKSDDTNHWHECSRCHDKKDEAAHSASEWIIDTAATETAEGAKHKECTVCKKVLETATIPATGSSHTHSYGVYVGMTYTAGNLIYQITSIDTATLGQSKVIGVVAAKKNKITKITIPDRADCKGYRLNVTTIGNNAFAGCKALKKLTIGNKVTVIGKNAFKKCSKLKTVVIGKAVKTISSKAFIGDNKIKKITFKGKKLKTVNKNAFSKKAKKNIKSKKTKLKGNKKAIKLFKKKLKIK

SEQ ID NO: 64 - protein, 1139 aa, Coprococcus eutactus
MTKKITAIFLALCMAISVLPMTIQAASKPDIKVGDYVKMGAYNNASILWRCVSIDNNGPLMLADKIVDTLAYDAKTNDNSNSKSHSRSYKRDDYGSNYWKDSNMRSWLNSTAAEGKVDWLCGNPPKDGYVSGVGAYNEKAGFLNAFSKSEIAAMKTVTQRSLVSHPEYNKGIVDGDANSDLLYYTDISEAVANYDSSYFETTTEKVFLLDVKQANAVWKNLKGYYVAYNNDGMAWPYWLRTPVTDCNHDMRYISSSGQVGRYAPWYSDLGVRPAFYLDSEYFVTTSGSGSQSSPYIGSAPNKQEDDYTISEPAEDANPDWNVSTEQSIQLTLGPWYSNDGKYSNPTIPVYTIQKTRSDTENMVVVVCGEGYTKSQQGKFINDVKRLWQDAMKYEPYRSYADRFNVYALCTASESTFDNGGSTFFDVIVDKYNSPVISNNLHGSQWKNHIFERCIGPEFIEKIHDAHIKKKCDPNTIPSGSEYEPYYYVHDYIAQFAMVVNTKSDFGGAYNNREYGFHYFISPSDSYRASKTFAHEFGHGLLGLGDEYSNGYLLDDKELKSLNLSSVEDPEKIKWRQLLGFRNTYTCRNAYGSKMLVSSYECIMRDTNYQFCEVCRLQGFKRMSQLVKDVDLYVATPEVKEYTGAYSKPSDFTDLETSSYYNYTYNRNDRLLSGNSKSRFNTNMNGKKIELRTVIQNISDKNARQLKFKMWIKHSDGSVATDSSGNPLQTVQTFDIPVWNDKANFWPLGALDHIKSDFNSGLKSCSLIYQIPSDAQLKSGDTVAFQVLDENGNVLADDNTETQRYTTVSIQYKFEDGSEIPNTAGGTFTVPYGTKLDLTPAKTLYDYEFIKVDGLNKPIVSDGTVVTYYYKNKNEEHTHNLTLVAAKAATCTEGGKEAYYKCEGCGKFYEDVLGTKEITDLASWGNIAKIAHTTKQTVTKATPTANGKIVNYCSVCKKTLSTTVIPKASSIKLKATSLTYNGKVRTPKVIVKDRTGKTLVKNTDYTVSYAKGRKYVGKYAVKITFKGKYSGTKTLYFTIKPKATSISSLKAGSKKFTVKWKKQATQTTGYQVQYSASSKFSKAKTVTVGKNTTVSKKISKLSGKKKYYVRVRTYKTVKINGKSIRIYSGWSKAKTVTTKK

SEQ ID NO: 65 - protein, 1331 aa, Coprobacillus cateniformis
MTKKITAIFLALYMAISVLPMTIQAASKPDIKVGDYVKMGVYNNASILWRCVSIDNNGPLMLADKIVDTLAYDAKTNDNSNSKSHSRSYKRDDYGSNYWKDSNMRSWLNSTAAEGKVDWLCGNPPKDGYVSGVGAYNEKAGFLNAFSKSEIAAMKTVTQRSLVSHPEYNKGIVDGDANSDLLYYTDISEAVANYDSSYFETTTEKVFLLDVKQANAVWKNLKGYYVAYNNDGMAWPYWLRTPVTDCNHDMRYISSSGQVGRYAPWYSDLGVRPAFYLDSEYFVTTSGSGSQSSPYIGSAPNKQEDDYTISEPAEDANPDWNVSTEQSIQLTLGPWYSNDGKYSNPTIPVYTIQKTRSDTENMVVVVCGEGYTKSQQGKFINDVKRLWQDAMKYEPYRSYADRFNVYALCTASESTFDNGGSTFFDVIVDKYNSPVISNNLHGSQWKNHIFERCIGPEFIEKIHDAHIKKKCDPNTIPSGSEYEPYYYVHDYIAQFAMVVNTKSDFGGAYNNREYGFHYFISPSDSYRASKTFAHEFGHGLLGLGDEYSNGYLLDDKELKSLNLSSVEDPEKIKWRQLLGFRNTYTCRNAYGSKMLVSSYECIMRDTNYQFCEVCRLQGFKRMSQLVKDVDLYVATPEVKEYTGAYSKPSDFTDLETSSYYNYTYNRNDRLLSGNSKSRFNTNMNGKKIELRTVIQNISDKNARQLKFKMWIKHSDGSVATDSSGNPLQTVQTFDIPVWNDKANFWPLGALDHIKSDFNSGLKSCSLIYQIPSDAQLKSGDTVAFQVLDENGNVLADDNTETQRYTTVSIQYKFEDGSEIPNTAGGTFTVPYGTKLDLTPAKTLYDYEFIKVDGLNKPIVSDGTVVTYYYKNKNEEHTHNLTLVAAKAATCTTAGNSAYYTCDGCDKWFADATGSVEITDKTSVKIPAPGHTAGTEWKSDDTNHWHECSRCHDKKDEAAHDYGSDNVCDTCGYYKTVPHTHNLTLVAAKAATCTTAGNSAYYTCDGCDKWFADATGSVEITDKTSVKIPAPGHTAGTEWKSDDTNHWHECTVAGCGVIIESTKSAHTAGEWIVDTPATATTAGTKHKECTVCHRVLETQPIPSTGTELKIIAGDNQIYNKASGSDVTITCNGDFAKFTGIKVDGSVVDSSNYTAVSGSTVLTLKASYLGTLTDGSHTITFVYTDGEANANLTVRTAGSGHIHDYGTEWKSNADNHWHECNCGDKKDEAAHSFKWVVDKEATATKKGSKHEECKICGYKRSAVEIPATGTSTAPTDTTKPNDTTKPGNTNGSEKSPQTGDNSNIFLWFALLFVSAAGVTGITAYNKKKKEHAE

SEQ ID NO: 66 - protein, 1276 aa, synthetic construct
MTKKITAIFLALCMAISVLPMTIQAASKPDIKVGDYVKMGAYNNASILWRCVSIDNNGPLMLADKIVDTLAYDAKTNDNSNSKSHSRSYKRDDYGSNYWKDSNMRSWLNSTAAEGKVDWLCGNPPKDGYVSGVGAYNEKAGFLNAFSKSEIAAMKTVTQRSLVSHPEYNKGIVDGDANSDLLYYTDISEAVANYDSSYFETTTEKVFLLDVKQANAVWKNLKGYYVAYNNDGMAWPYWLRTPVTDCNHDMRYISSSGQVGRYAPWYSDLGVRPAFYLDSEYFVTTSGSGSQSSPYIGSAPNKQEDDYTISEPAEDANPDWNVSTEQSIQLTLGPWYSNDGKYSNPTIPVYTIQKTRSDTENMVVVVCGEGYTKSQQGKFINDVKRLWQDAMKYEPYRSYADRFNVYALCTASESTFDNGGSTFFDVIVDKYNSPVISNNLHGSQWKNHIFERCIGPEFIEKIHDAHIKKKCDPNTIPSGSEYEPYYYVHDYIAQFAMVVNTKSDFGGAYNNREYGFHYFISPSDSYRASKTFAHEFGHGLLGLGDEYSNGYLLDDKELKSLNLSSVEDPEKIKWRQLLGFRNTYTCRNAYGSKMLVSSYECIMRDTNYQFCEVCRLQGFKRMSQLVKDVDLYVATPEVKEYTGAYSKPSDFTDLETSSYYNYTYNRNDRLLSGNSKSRFNTNMNGKKIELRTVIQNISDKNARQLKFKMWIKHSDGSVATDSSGNPLQTVQTFDIPVWNDKANFWPLGALDHIKSDFNSGLKSCSLIYQIPSDAQLKSGDTVAFQVLDENGNVLADDNTETQRYTTVSIQYKFEDGSEIPNTAGGTFTVPYGTKLDLTPAKTLYDYEFIKVDGLNKPIVSDGTVVTYYYKNKNEEHTHNLTLVAAKAATCTTAGNSAYYTCDGCDKWFADATGLVEITDKTSVKIPALGHTAGTEWKSDDTNHWHECSRCHDKKDEAAHDYGSDNVCDTCGYYKTVPHTHNLTLVAAKAATCTTAGNSAYYTCDGCDKWFADATGLVEITDKTSVKIPALGHTAGTEWKSDDTNHWHECSRCHDKNDEAAHSTSEWIIDTAATETAEGAKHKECTVCKKVLETATIPATGSSHTNSYGVYVGMTYTAGNLIYQITSIDTATVGQSKVIGVVAAKKNKIKKVTIPDRADCKGYRLNVTTIGNNAFAGCKALEKLTIGNKVTVIGKNAFKNCSKLETVVIGKAVKTISSKAFIGDNKIKKITFKGDKLKTVKKNAFSKKAKKNIKSKKTKLKGNKKAIKLFKKKLKIK

SEQ ID NO: 67 - protein, 1329 aa, Clostridiales bacterium
MKKYFEKTSIALIIAMMFILAIFGGEAMKTHTIDDITKYKMVVNAQGVKTENGTRTTTQVELGNYISLGKYNGKEILWRCVGEDENGALMLADNIIDTLPYDAKTNDNNRSKSHSRNYKRDTYGSNYWKDSNMRSWLNSTAVAGEVKWLCGNPPREDSVNGNAYDQKAGFLNDFSKAEIAAMKNVTQRSIVSHPEYNLGFHDGEGRSDLELNFDIENVASNFDSAYGENSTEKVFLLDVKQVNTVWKNFGNYYIGRNEQGMAWPYWLRTPVTDCNHDMRYVHSNGSVGREWPNTDYIGVRPAFYLDSDYYATTSGDGSASNPYVGSAPDKIEDDYTVAEPEEDPNQEWDISLDQQLRLTLGPYYSSDGKYATPTIPVYTIQKTRSDTENMVILICGEGYTKSQQQKFIDDVKKVWEGAMQYEPYRSYADRFNVYALCTASESNFNSGGSTFFDVVIDKKSGPMISVNKSAWKNHIFERCIGPTFLEQIHDAHIPNKTDPDTFIWDDDKMYPPFYYVHKYINQFAVLVNTTQDFGGSHRNYKRGIHYLITPADSPRAQKTFTHELGHGLLELGDEYMTTAAESTDYTSLNVAYTHDPEKVKWKQMLGFRKTFTCNTSPSYTAYNSSWECLMRDTTYQFCEVCKLQGSKRMSQLIDGKSLYVADPEVKKYTVQYSKPSDFADTTYNGYYYFENYRNNVLLSGVDKNKFNTSMAGEKIQLRTIVQNLSDTTQRYVTMKLWIKHAGGSVATTTGGQRLEATQTFTIPVWSEKSKFWPKGALSYEGSNMNSGLENCELIYQIPLDADLKHGDYVAFEVTDESGNILANDNTETQTYANINIEYKFEDGTPMPNANKATIPVAVGSQLNWTAPSTMFGHTFVRAEGHDQMVNGSGQTVTYYYTKQSNVHIHDWGEVKYTWTSDNTCKAERVCKHDSTHIESETVTATGTTITAATCKEKGKMKYTATFVNTAFSMQEKEVDIDFAEHTYGAWIEEVPATCIAGGMKAHYKCTVCGKYFDENKNETTEEALKTPVSPYYGHSFGFWVEEQYATCQAPGRKGYKHCSICNKDYDASNTEITDFVIPINPDGHELGDLVAEVPATCKDTGVKEHRDCRLCGKHCDPITRKEIADLTIPTTNNHTYGELIPEVSPTTTEFGVKEHKDCTVCGRHFDKDGNEITELRIAKIGTHNVIVNGESKFYAHGESVTVTANEPAEGKVFKGWQDASGKIVSTDKSYTFTVNGETTLTAVYEDKSSGGGEITPPAKKDGLSGGQIAGIVTGSAAVAGLGGFAVLWFVVKKKTFADLGALLKKGFTAIGNFFKTLGEKIKALFTKKK

SEQ ID NO: 68 - protein, 1336 aa, Roseburia faecis
MKKQLTALVLCICMVLSVLPFSSTQAAAEETSSVGTSNISIGDYIRLGNYNGQPILWRCVDVDEMGPLMLSDQVLATMAYDAKTSENSATRSHSRNLKRGTYGSNQWRDSNMRSWLNSKAEAGKVEWLCGNPPKSGFVGENPYDQAAGFLNGFKEDEIAAIKTVTQRSIVSHPEYNAGMIEGQGADLPYDTNIEAAANGFDQAYYENVTDKVFLMDVKQINKVYQNNSQLGGSYHIAYKGGVRWPYWLRTPVTDCNHDMRYVETDGRIDRNAPYLGFYGVRPAFYLDTQYYQVTGGDGTADSPYRGAAVNKPEENFTVSGDGPTPGQEWDVSLDKSIQLYLGPNYSKSKKYESATIPIQVIQKTRSDNENMVVVICGEGYTKGEQQKFVAAAKRLWEGAMQYEPYKTYKDRFNVYALCTASDKTYSAIDGYDSTFFDVWGKNISVNGSQWKNHIFERCIGPAFIEKVHDAHIPQQADPNVDWDFEKYKYVHDYISQFVLLVNSANDFGGAFNDLDYGFHYIVSPAYSQRAVETLTHELGHGLLWLGDEYNSGSFMGEASEKTSLNRTGISDPEQVKWRQLLGFRKTYSVPHTDYDTDKIYNSSRECMMRQTWNGFCEVCKLQGNKRMRQLVTEGPDLYVAEPEVTKRTDAYTKLSDFSDATGWGYTKFDADKKTRLLTGADKITFQPTEMKGQKIELRTIVQNLSDTKLSQVTLQVWVNHADGTIATADGQPVAASETFKIPLWTEKGNFRPKGTLEYHGSDFNSGLKNCSLLYTIPSNADLRTGDTVGYAVRDEQGTVLAYEGTLPNKGQDILPAPEPAKSYTVTFCYNDGRENTTKTTGINGKLGDLPAPAREGYVFDGWYTTGGEKVDLTRVYSSNTVLYARWSEYIAPSPNVKKAPVILLAASPDTVTEGEQVMLSVSETSGFGVDLSGVTYTADPSLPISGTGEAQTIRLDQAGTYTFTAHYSGDNEKYLAADSNRVTVTVTKKADVSGGTTSGGGSSSGGGSTAGGGSSAGGGSSAGGGSSSGGGAAGGATAGGGAANGNASATTTPDIKDSDGTTVAIVNGKKGMITAEVQLSEKAIANAEKSGEAVKLPVEVKAGKNIKAASTVTINLPEGAGKTKVKIPVKNMTAGTVAVLVNADGTEKIVKKSVAAKDGVQLIVDEDTTVKLVDKAKNFKDTKKHWAKDSIDFVSARGLMNGKSSTAFAPEAKITRARLWTILARWEDVDLTGGKKWYSKARAWAKNQGISDGSRPNAAITRAEAITMLWRAQGKPAAEQETAFKDVSSDEYYAQAVAWAKEKGIAQANSKGRFNPDAACTRAEIAAFLYRMSLSE

SEQ ID NO: 69 - protein, 1153 aa, Clostridium sp.
MKKNFGKASIALIIAMMFILAFFGGDVMKAHTIDGSASNLYVGSALDKVEDDYTVAEPEKAPNQELDISIEQSLNLTLGEWYSSDGKYANPTIPVYTIQKTRSDTENMVILICGEGYTKNQQQKFVNDVKKVWEGAMQHEPYRSYADRFNVYALCTVSESSFNSGGSTFFDVVIDKNSGPMIAISKSICKNHIFERCIGPAFLEQIHDVHIPKKVDPNSSYWVGNNSPLSEYEPFYYVHEYINQFAILVNTTQDFGGSHRNYERGIHYLVTPADSDRAQKTFTHELGHGLLELGDEYMSSTTQQTDLTSLNVAHTHDPNNVKWKQLLGFRKTYTCNALGYGNAYNSSYECLMRDTAYQFCEVCKLQGSKRMSQLIDGKSLYVAVPEVKKYTGQYSKPSDFIDTTYNGYYYFENYRKGVLLSGTDKNKFNTSMAGETIQLRTIVQNLSDTKQRYVTMKLWIKHADGSVATTTGGQRLEATQTFTIPVWSEKSKFWPKGALSYEGSHMNSGLENCELIYQIPSDAVLNNGDTVAFEVIDENGNILANDNTETQAYANINIEYKFEDGTPMPNVNQAMIPVAVGSQLNWTAPSTMFGHKFVRAEGHDQMVNGSGQTVTYYYKKQSNVHIHDWGEVIYTWISDNICKAERVCKHDSAHIESETITATGTVIKASTCTEKGKVKYTARFTNTAFGVQYREVDIDLVEHKFGEWIDEIPATTENFGTKGHKDCTVCKKHFDKDGNEITDLRIAKISTYTVTVKDGADETNTHYKSGDTVTIKVTIPTGKHFVKWSAVTGISLSASQLTQEEITFTMPDNDVTLIAELEDILYRVTVIGGTTTLNEAKYQENVTVTANTPEVGKEFDKWIVSGITLSNTNLTRSTLTFTMPENDVTFTATYKDIVYRVMVEEGKATPEMAIYQTEVTVMANEPAIDMYFDKWEVMGLDTTGMDLTKTQIKFQMPAGNVTFKATYLPHIKYGILVVDGTKDKSPVMAGEIVTITANPAKPGKVFDKWTCETVGVTIEFASATSKQTTFVMPAQDIKIKAHFKDIEVAPSVEIKVEGGTGAGTYKPGDSVTITANEPAEGKVFKCWKDEKGEIVSTDRSYAFIVNGETTLTAVYEDKASGGAIAGIVIGSILGVGIIGFVIFWFAVKKKDVF

SEQ ID NO: 70 - protein, 1158 aa, Acholeplasmatales bacterium
MRWNIMKKYFGKANIALIIAMMFILAFFGGEAMKTHTIDGSASNLYVGSALDKVEDDYTVAEPEKAPNQELDISIEQSLNLTLGEWYSSDGKYANPTIPVYTIQKTRSDTENMVILICGEGYTKNQQQKFVNDVKKVWEGAMQHEPYRSYADRFNVYALCTVSESSFNSGGSTFFDVVIDKNSGPMIAISKSICKNHIFERCIGPAFLEQIHDVHIPKKVDPNSSYWVGNNSPLSEYEPFYYVHEYINQFAILVNTNQDFGGSHRNYERGIHYLVTPADSDRAQKTFTHELGHGLLELGDEYMSSTTQQTDLTSLNVAHTHDPNNVKWKQLLGFRKTYTCNALGYGNAYNSSYECLMRDTAYQFCEVCKLQGSKRMSQLIDGKSLYVAVPEVKKYTGQYSKPSDFIDTTYNGYYYFENYRKGVLLSGTDKNKFNTSMAGETIQLRTIVQNLSDTKQRYVTMKLWIKHADGSVATTTGGQRLEATQAFTIPVWSEKSKFWPKGALSYEGSHMNSGLENCELIYQIPSDAVLNNGDTVAFEVIDENGNILANDNTETQAYANINIEYKFEDGTLMPNVNQAMIPVAVGSRLNWTAPSTMFGHKFVRAEGHDQMVNGSGQTVTYYYKKQSNVHIHDWGEAIYTWTSDNICKAERVCKHDSAHIESETITATGTVIKAATCTEKGKVKYTARFTNTAFGVQYREVDIDLVEHKFGEWIDEIPATTENFGTKGHKDCTVCKKHFDKDGNEITDLRIAKISTYTVTVKDGADETNTHYKSGDTVTIKVTIPTGKHFVKWSAVTGISLSASQLTQEEITFTMPDNDVTLIAELEDILYRVTVIGGTTTLNEAKYQENVTVTANTSEVGKEFDKWIVSGITLSNTNLTRSTLTFTMSENDVTFTATYKDIVYRVMVEEGKATPEMAIYQTEVTVMANEPAIDMYFDKWEVMGLDTTGMDLTKTQIKFQMPAGNVTFKATYLPHIKYGILVVDGTKDKSPVMAGEIVTITANPAKPGKVFDKWTCETVGVTIEFASATSKQTTFVMPAQDIKIKAHFKDIEVAPSVEIKVEGGTGAGTYKPGDSVTITANEPAEGKVFKCWKDEKGEIVSTDRSYAFTVNGETTLTAVYEDKASGGAIAGIVIGSILGVGIIGFVIFWFAVKKKDVF

SEQ ID NO: 71 - protein, 1557 aa, Clostridiales bacterium
MILLQIYYTKEGVKMKNKQINRTLSLLLSVVMVLSLCPLIAKAEGTKPNIKIGDYIKLGTYENEPILWRCVDIDDNGPLMLMDKVLGSMPYDAKTSENSATRSHSRNSFRSSYGSNHWRDSNMRSWLNSDADAGKVDWLCGNPPKSDYVGYGSEYDKKAGFLNGFSKAEIAAIKTVTQRSIVSHPEYSAGYIAGPGADLPYNTDIASVAYGFEKAYYENIIDKVFLPDVKQLNTIYNNSNILGNYYLAKNKDGIRWSYWLRTPITDCNHDMRYVETDGNIYRVAPYFGHIGVRPAFYLDTDYYIVSEGNGEVNSPYVGDAADKPGDDISISGPDEEGGDGDWDIDTDQSIQLNLGPWYSSDGEYANSTIPVQVIQKTRSDLENMVIVICGEGYTKDQQQKFINDVKRIWAGVLKHEPYRSMADRFNVYALCTASKTSGFASENTFFDITMSTTSRSPMISLYKSVLKNQILTRCIGPAFIEKIHDAHIKEKTNPNEITIGDEYAPYYYVNEYISQFVVLVNSGQYGGASMNNLDVGLHYVTATVDNIQSEYTLAHELGHGLLHLGDEYNAYGGAYTMPEQQDKQSLNIAGLRESPITIKWKDMLGFRKTYTCRDSNTSNSSNMVNSSWQCMMRTQNQELCDVCQLQGFKVMSQLIKDTDDIYIAIPEVKLYTGNYKNPFEDYSAYTEAEYYGYLAYASDRAQRLLSGTSKNKFTKDMKGQEVELRTIAQNLSGIEEQEITLQLWVEHEDGTRAVTENGEEILKEQTFTVPVWDEKENFYIKGMRNYSGTEFDSGLMNCSLIYKIPENADLKDGDTIKFSVIDKMGKTLADDNTETQNYANVTISYQLEDSNAVPNTQTAVIPVPIGTKMDIEPPGELYGYKFVKAEGLGKIVGDDGLNIICYYEDPSGKLPVEYKVEYDWGTDFPTDTTLPTDNTKYDSIENAKESVKNQKYDENSTSTVKKNDKDGTWTFSGWTATVEGTTVKFTGAWTFTATPIITYTVTYDWGTDFPTGEMLPVDSKTYKSEEDAKAAMDGKYTSLSTSTAEKDGKSGTWKFSGWIATLIGTTVKFNGMWTFTPDAPVVDADTPTNIKLVSDEYKIGDKATALDGKATVSDNGVLSYQWYKSDKADNFNGTAIDGQNGETFVPDTSKEGTYYYYVIATNTKADATGKKTASVTSSMAIIHVKESVKYTVVYDWGSDYPTDVTVPKDDTKYENIEKAKEAVKNQKYDENSTSTAEKNSKSGKWSFSGWTTAVEGTTVKFTGVWTFTENAIPVVTRKPSSGGSGGSGSSTYNIKVSPEITNGSLSVNPSRASNGKKVSVIVKPNNGYVLNSVIVKDSNDKEIAVTKQSDGTYTFIMPSSNVTVSAKFDTELAKDVVTEIEKSIEFKDVKKGDWYFDAVQWAVKNNITEGSGKDTFSPDVICTRTQMVTFLWRVAGSPEPKITKCDFRDVDNSAYYYKAVLWAVEKGVTVGTSDTTFSPNENVTRGQTVAFLYREAGSPFETGEDVFNDVNSNDYYFKAVSWATKNGITVGTGNGKFEPDMDCNRAQIVAMLYRTQR

SEQ ID NO: 72 - protein, 1188 aa, Clostridium sp.
MKKHLKKTSIALTIVMMFIPAIFGGKAITIHTNADNTNYKTAVNAQGVKTEKETKATTQVELGNYISLGKYNGNEVIWRCVSIDEKGALMLADNIIDTLPYDAKTNDNNHSKSHSRNNNRDNHGSNYWKDSNMRSWLNSTAVAGEVTWLCGNPPRAGYLNENAYDQKAGFLNDFSKAEIALMKNVTQRSLVSHPEYNHGFHDGDGHSDLEFNENIENVSSNFNSAYGENSTEKVFLLDVQQVNKVWENFDNYYIGRKEGVAWPYWLRTPLSSCNHLMRYVGSNGLVGKDYPTNAIGVRPAFYLDSDYYVTTSGNGSASNPYVGSAPDKIEGDYIIAEPEEDPNQEWDVSLDQQLRLALGPYYSSDGKYSTPTIPVYTIQKTRSDTENMVILICGEGYTKSQQQKFINDAKKVWEGAIQYEPYRSYADRFNVYALCTASESSFNNSGSTFFDVVIDKKVGPMISVNKSSWKNHIFERCIGPAFIEQIHDAHIPNKTDPDTFIWDDDKMYSPFYYVHKYINQFALLVNTSQDFGGSHRNYKRGIHYFITPADNNRAVKSFAHELGHGLLELGDEYMTVAAESTDYTSLNVAYNHNPEQVKWKKLLGFRKTFTCNTYPFYTAYNSSWECLMRDTNYQFCEVCKLQGYKRMSQLIDGKNLYVADPEVKKYTDRYTNPSDFAETNYNGYINFTNYRDEILLSGWNKNKFNTGMVGEKIQLRTIVQNLSDTTERQVTMKLWIKHADGSIATTTNSQRLEATQTFTIPVWSEKSKFWPKGALEYNGSNLNSGLENCELIYQIPSDAVLNNGDTVAFEVTDENGNVLAHDNTETQPYANVNIEYKFEDGSPMPNANKAVIPLAVGSYINWTAAPSLYGYALSRVEGLNQIVSGSDQTVTYYYTKKIGTHIHDWGDWVSNGDGTHTRTCTKDSSHTETENCSGGTATCTTKAVCSVCGFTYGEKLGHNWGEVKYTWMSDNICKAERVCKHDSTHIESEMVTATGTVITKATCKEKGKMKYTATFVNTAFTVQEKEIDTDFAPHTFGAWKDEIPATTEEFGTKGHKDCMDCGRHFDKDGKEITELRIAKIGTYNVVINGESKFYADGESVTVKAEDKEGKIFKGWQDESGEIVSTEKSYTFTVTGDRSLTAVYENVLATKKGLSDRQIAGIIIGSVVAAGLGGFAIFWFVIKKKGLRL

SEQ ID NO: 73 - protein, 1334 aa, Lachnospira eligens
MNIIKHKYGKRTVSLLLAVILVLCPLPVRAADNKPTIEIGDYIQMGTYGGVPIVWRCVAKDSNGPLMLSDRVLCDYMPYDAKTNKNAETGSHRRNSWRDNFGSNHWRDSNIRSWLNSNAEAGKVKWLCGNPPTEDSVYPKTAAYDQKEGFLRSFRSDELGAIRTVKQRSIVSHPEYTAGYIDAAGVDLLYNTTIDTVADGYDSAHYEYIWDRVFLLDVQQLKTVNDNLNGYHIAKNRSGVAWNYWLRTPITTCNHDMRFVTPQGNILRDAPYKGYYGVRPAFYLNTENYTVSSGTGQSAQDPYVVSAPDATDDSIGISGAVREDVNGDWNVNTDEYLQLEMSTLYTEDPAYANVTVPVYTIQKPRSDKENMVIVYCAEGYTKSQQKQFVEDVKKLWGEVLQIEPYRSMADRFNVYALCTASVDGYGGTSTFFAATAKGGISTNKGNWRNHVLERIIGPAFIEKIHDAHIPNETHPNENTMDHNYRQYDYVYENINQFVVLANSGEYFGGSHDNKQYGIHYIVASARNAYSAFTQRHELGHGLFHLGDEYNYSTVPVDEWNYTTSLNMTATKDPTKVKWKQLLGFRNTYTCPHLDYYPYTYNSSRDCLMRETFQNDFCDVCKLQGIKVMSQLITNPPALYVAVPEVKKYIGGYRNPTKDPSAFEAANSSAYASYQNDRNSRLLSGGSKNSFDYSSMKGQQVELRTIIQNLSNTQAKTVTLRLWVEHSNGEKAVTTDGEQVFTTQEFDIPVWKEKSKFWTKGALDYEGSDFNSGLVNCSLVYTIPENAILQSGDTIGFEIVDHATGEVLADDDTEQQRYVNVTIQYQLEDGTDVPNTMPTTFTVPVGKKVDWQPPQELHGYTFVKAEGMENAVPNSGMTIRYIYKRSEERPEPPVTKNYTVQYNWGSVFPTGATLPLNSSSYSSVQQAKAAVDKKYTSTTRIQAQKDGKNGTWAFSGWDAGNLNGTTVVFRGSWSFTADTAPITPPSGTASYKITATAGIGGTISPGGTTTVSAAGQLTYTIKANEGYYIADVKVDGSEVTATTSYTFSDVNTDHTIEVTFKQESQTPDVPDVIAPSITTQPGNATVKVGETASFTIAASGTDLTYQWQIDRNDGKGWVNIDGATATSYTTSTVNISCNGFKYKCVVSNSAGNVESNSATLTVQDAGGSDNPDTPNNTYQIIDGANSSWTHDSDGNITIRGNGDFSKFTGVKVDGNLIDKSNYTAKEGSTIITLKASYLNTLSAGNHTVEILWTDGSASTTFTTKANISDNSNNNQNDNNNSNSSDDKPSSGTDKKDVTAPKTGDNTPSVWLFILSILSGTGLIITVKKRRENLNS

SEQ ID NO: 74 - protein, 842 aa, Dorea longicatena
MNVIKHRYGKRTVSLLLAVILVLCPLRVRAADNKPTIGIGDYIKSAQDPYVVSAPDAPDYSIGISGAVRDDVNGDWNVNTDEYLQLKMSTYYTEDTAYANVTVPVYTIQKPRSDKENMVIVYCAEGYTKSQQKQFIEDVKKLWGEVLQIEPYRSMADRFNVYALCTASVDSFGGTSTFFNATKKGISNSKGAWRNHILERIIGPAFIEKIHDAHIPNKTHPNENPGDHDYRQYDYVYENINQFVLLANSGEYFGGSHDNKEHGIHYIIASARSQYSAFTQRHELGHGLFHLGDEYNYSTVPVAEANYTTSLNMTATKDPTKVKWKQLLGFRNTYTCPHDDRYPYTYNSSRDCLMRETFQNDFCDVCKLQGIKVMSQLITNPPALYVAVPEVKKYIGDYRNPTEKPSAFEAANSSAYASYQYDRNSRLLSGGSKNSFDYGSMKGQQVELRTIIQNLSDTQAKTVTLRLWVEHSNGEKAVTTEGQQVFATKDFAIPAWSEKSKFWPKGALDYKGSDFDSGLVNCSLVYTIPENATLQYGDTIGFDIVDRATGEVLAHDDTEKQPYADVTIQYQLEDGTDVPNTMPTTFTVPVGKKVDWQPPQELNGYTFVQAEGMEETVPSNGMTIRYIYKRTEERPEPPVTKNYTVKYDWGSVFPTGVTLPQNSNSYSSEQQAKAAVDKKYTTSTRIKAQKDGKNGTWAFSGWDSGSLNGTTVVFRGSWSFTADTAPITPPSGGGGGGGAATTASYKITATAGIGGTISPGGTTTVSAAGQLTYTIKANEGYYIADVKVDGKSVGAVSSFAFEKITASHTIEASFAKKDSATVKDPIKRLPIHLPIKMKVKKM

SEQ ID NO: 75 - protein, 951 aa, Clostridium sp.
MKKTYLFKSYKRKSQKEVEHNEKNILKKTIIALIIAMMFILAIFFGGEAMKTHTIDDVAKYKMVVNAQGVKMGNGTRTQTQVDLGNYISLDQQLKLTLGPYYSSDGKYSTPTIPVYTIQKTRSDTENMIILICGEGYTKSQQQKFIEDVKRVWDGAIQHEPYRSYADRFNVYALCTASESSFNSGGSTFFDVVIDKKSGPRISGNKSAWKNHIFERCIGPTFLEQIHDAHIPNKTDPDTFIWDDDKMYPPFYYVHKYINQFAVLVNTEQDFGGSHRNYKSGIHYLITPADSPRAQKTFTHELGHGLLELGDEYMTSATESTDYTSLNVAYTHDPEKVKWEKMLGFRKTFTCHTNSSYTAYNSSWECLMRDTTYQFCEVCKLQGSKRMSQLIDGKSLYVADPEVKKYTGQYSQPSDFADTTYNGYANFSYYRSGVLLSGWDKNKFNTDMAGEKIQLRTIVQNLSDTTQRYVTMKLWIKHADGSVATTTGGQRLEATQTFTIPVWSEKSKFWPKGALSYEGSNMNSGLENCELIYQIPLDAVLNKGDTVAFEVTDENGNVLANDNTETQTYANINIEYKFEDGTPMPNVNKATIPIAVGSKLNWTAPSTMFGHTFVRAEGHDQMVNGSDQTVTYYYAKQSNVHIHDWEEWVSNGNGTHTRTCRTDNSHSETANCVGGTATCTHKPVCEVCHGEYGQAKSHDWGKATYTWTDTVCKAERVCKHDSAHTESETRTATGTVIKAATCKEKGKMKYTATFENTAFTKQEKKVDINFAGHTFGKWQDEIPATTEAFGTKGHKDCSVCGRHFDKDGNEITELRIAKIVTHNVIVNGESKFYAHGESVTVTANEPAEGKVFKGWQDASGKIVSTKKSYTFTVNGETNLTAVYEDKTSGGEIVPPAKKDGLSGGQVAGVVIGSAAVAGIGGFAIFWFTVKKKTFADLIAAIKSLFTKKKTK

SEQ ID NO: 76 - protein, 1210 aa, Butyrivibrio crossotus
MNIIKHKYGKRTVSLLLAVILVLCPLQVRAADNKPTIEIGDYIQMGTYGGVPIVWRCVAKDSNGPLMLSDRVLCDYMPYDAKTNKNAETGSHRRNSWRDNFGSNHWRDSNIRSWLNSNAEAGKVKWLCGNPPTEDSVYPKTAAYDQKEGFLRSFRSDELGAIRTVKQRSIVSHPEYTAGYIDVAGVDLPYNTTIDTVADGYDSAHYEYIWDRVFLLDVQQLKTVNDNLNGYHIAKNRSGVAWNYWLRTPITTCNHDMRFVTPQGNILRDAPYKGYYGVRPAFYLNTENYTVSSGTGQSAQDPYVVSAPDAPDDSIGISGAVREDVNGDWNVNTDEYLQLEMSTLYTEDPAYANVTVPVYTIQKPRSDKENMVIVYCAEGYTKSQQKQFVEDVKKLWGEVLQIEPYRSMADRFNVYALCTASVDGYGGTSTFFAATAKGGISTNKGNWRNHVLERIIGPAFIEKIHDAHIPNETHPNENTMDHNYRQYDYVYENINQFVVLANSGEYFGGSHDNKQYGIHYIVASARNAYSAFTQRHELGHGLFHLGDEYNYSTVPVDEWNYTTSLNMTATKDPTKVKWKQLLGFRNTYTCPHLDYYPYTYNSSRDCLMRETFQNDFCDVCKLQGIKVMSQLITNPPALYVAVPEVKKYIGGYRNPTKDPSAFEAANSSAYASYQNDRNSRLLSGGSKNSFDYSSMKGQQVELRTIIQNLSNTQAKTVTLRLWVEHSNGEKAVTTDGEQVFTTQEFDIPVWKEKSKFWTKGALDYEGSDFNSGLVNCSLVYTIPENAILQSGDTIGFEIVDHATGEVLADDDTEQQRYVNVTIQYQLEDGTDVPNTMPTTFTVPVGKKVDWQPPQELHGYTFVKAEGMENAVPNSGMTIRYIYKRSEERPEPPVTKNYTVQYNWGSVFPTGATLPLNSSSYSSVQQAKAAVDKKYTSTTRIQAQKDGKNGTWAFSGWDAGNLNGTTVVFRGSWSFTADTAPITPPSGTASYKITATAGIGGTISPGGTTTVSAAGQLTYTIKANEGYYIADVKVDGSEVTATTSYTFSDVNTDHTIEVTFKQESQTPDNTYQIIDGANSSWTPDSDGNITIRGNGDFSKFTGVKVDGNLIDKSNYTAKEGSTIITLKASYLNTLSAGTHTVEILWTDGSASTTFTIKANTSDDKPSSGTDKKDDAPKTGDNTPSVWLFILSILSGTGLIITVKKRRENLNS

SEQ ID NO: 77 - protein, 229 aa, synthetic construct
ESKYGPPCPSCPAPEFLGGPSVFLFPPKPKDTLMISRTPEVTCVVVDVSQEDPEVQFNWYVDGVEVHNAKTKPREEQFNSTYRVVSVLTVLHQDWLNGKEYKCKVSNKGLPSSIEKTISKAKGQPREPQVYTLPPSQEEMTKNQVSLTCLVKGFYPSDIAVEWESNGQPENNYKTTPPVLDSDGSFFLYSRLTVDKSRWQEGNVFSCSVMHEALHNHYTQKSLSLSLGK

SEQ ID NO: 78 - protein, 10 aa, synthetic construct
GGGGSGGGGS

SEQ ID NO: 79 - protein, 15 aa, synthetic construct
GGGGSGGGGSGGGGS

SEQ ID NO: 80 - protein, 20 aa, synthetic construct
GGGGSGGGGSGGGGSGGGGS

SEQ ID NO: 81 - protein, 761 aa, synthetic construct
EYFVTTSGSGSQSSPYIGSAPNKQEDDYTISEPAEDANPDWNVSTEQSIQLTLGPWYSNDGKYSNPTIPVYTIQKTRSDTENMVVVVCGEGYTKSQQGKFINDVKRLWQDAMKYEPYRSYADRFNVYALCTASESTFDNGGSTFFDVIVDKYNSPVISNNLHGSQWKNHIFERCIGPEFIEKIHDAHIKKKCDPNTIPSGSEYEPYYYVHDYIAQFAMVVNTKSDFGGAYNNREYGFHYFISPSDSYRASKTFAHEFGHGLLGLGDEYSNGYLLDDKELKSLNLSSVEDPEKIKWRQLLGFRNTYTCRNAYGSKMLVSSYECIMRDTNYQFCEVCRLQGFKRMSQLVKDVDLYVATPEVKEYTGAYSKPSDFTDLETSSYYNYTYNRNDRLLSGNSKSRFNTNMNGKKIELRTVIQNISDKNARQLKFKMWIKHSDGSVATDSSGNPLQTVQTFDIPVWNDKANFWPLGALDHIKSDFNSGLKSCSLIYQIPSDAQLKSGDTVAFQVLDENGNVLADDNTETQRYTTVSIQYGGGGGSTCPPCPAPELLGGPSVFLFPPKPKDTLMISRTPEVTCVVVDVSHEDPEVKFNWYVDGVEVHNAKTKPREEQYNSTYRVVSVLTVLHQDWLNGKEYKCKVSNKALPAPIEKTISKAKGQPREPQVYTLPPSRDELTKNQVSLTCLVKGFYPSDIAVEWESNGQPENNYKTTPPVLDSDGSFFLYSKLTVDKSRWQQGNVFSCSVMHEALHNHYTQKSLSLSPGK

SEQ ID NO: 82 - protein, 761 aa, synthetic construct
TCPPCPAPELLGGPSVFLFPPKPKDTLMISRTPEVTCVVVDVSHEDPEVKFNWYVDGVEVHNAKTKPREEQYNSTYRVVSVLTVLHQDWLNGKEYKCKVSNKALPAPIEKTISKAKGQPREPQVYTLPPSRDELTKNQVSLTCLVKGFYPSDIAVEWESNGQPENNYKTTPPVLDSDGSFFLYSKLTVDKSRWQQGNVFSCSVMHEALHNHYTQKSLSLSPGKGGGGGSEYFVTTSGSGSQSSPYIGSAPNKQEDDYTISEPAEDANPDWNVSTEQSIQLTLGPWYSNDGKYSNPTIPVYTIQKTRSDTENMVVVVCGEGYTKSQQGKFINDVKRLWQDAMKYEPYRSYADRFNVYALCTASESTFDNGGSTFFDVIVDKYNSPVISNNLHGSQWKNHIFERCIGPEFIEKIHDAHIKKKCDPNTIPSGSEYEPYYYVHDYIAQFAMVVNTKSDFGGAYNNREYGFHYFISPSDSYRASKTFAHEFGHGLLGLGDEYSNGYLLDDKELKSLNLSSVEDPEKIKWRQLLGFRNTYTCRNAYGSKMLVSSYECIMRDTNYQFCEVCRLQGFKRMSQLVKDVDLYVATPEVKEYTGAYSKPSDFTDLETSSYYNYTYNRNDRLLSGNSKSRFNTNMNGKKIELRTVIQNISDKNARQLKFKMWIKHSDGSVATDSSGNPLQTVQTFDIPVWNDKANFWPLGALDHIKSDFNSGLKSCSLIYQIPSDAQLKSGDTVAFQVLDENGNVLADDNTETQRYTTVSIQY

SEQ ID NO: 83 - protein, 1413 aa, synthetic construct
EPKSCDKTHTCPPCPAPELLGGPSVFLFPPKPKDTLMISRTPEVTCVVVDVSHEDPEVKFNWYVDGVEVHNAKTKPREEQYNSTYRVVSVLTVLHQDWLNGKEYKCKVSNKALPAPIEKTISKAKGQPREPQVYTLPPSRDELTKNQVSLTCLVKGFYPSDIAVEWESNGQPENNYKTTPPVLDSDGSFFLYSKLTVDKSRWQQGNVFSCSVMHEALHNHYTQKSLSLSPGKGGGGGGGSASKPDIKVGDYVKMGVYNNASILWRCVSIDNNGPLMLADKIVDTLAYDAKTNDNSNSKSHSRSYKRDDYGSNYWKDSNMRSWLNSTAAEGKVDWLCGNPPKDGYVSGVGAYNEKAGFLNAFSKSEIAAMKTVTQRSLVSHPEYNKGIVDGDANSDLLYYTDISEAVANYDSSYFETTTEKVFLLDVKQANAVWKNLKGYYVAYNNDGMAWPYWLRTPVTDCNHDMRYISSSGQVGRYAPWYSDLGVRPAFYLDSEYFVTTSGSGSQSSPYIGSAPNKQEDDYTISEPAEDANPDWNVSTEQSIQLTLGPWYSNDGKYSNPTIPVYTIQKTRSDTENMVVVVCGEGYTKSQQGKFINDVKRLWQDAMKYEPYRSYADRFNVYALCTASESTFDNGGSTFFDVIVDKYNSPVISNNLHGSQWKNHIFERCIGPEFIEKIHDAHIKKKCDPNTIPSGSEYEPYYYVHDYIAQFAMVVNTKSDFGGAYNNREYGFHYFISPSDSYRASKTFAHEFGHGLLGLGDEYSNGYLLDDKELKSLNLSSVEDPEKIKWRQLLGFRNTYTCRNAYGSKMLVSSYECIMRDTNYQFCEVCRLQGFKRMSQLVKDVDLYVATPEVKEYTGAYSKPSDFTDLETSSYYNYTYNRNDRLLSGNSKSRFNTNMNGKKIELRTVIQNISDKNARQLKFKMWIKHSDGSVATDSSGNPLQTVQTFDIPVWNDKANFWPLGALDHIKSDFNSGLKSCSLIYQIPSDAQLKSGDTVAFQVLDENGNVLADDNTETQRYTTVSIQYKFEDGSEIPNTAGGTFTVPYGTKLDLTPAKTLYDYEFIKVDGLNKPIVSDGTVVTYYYKNKNEEHTHNLTLVAAKAATCTTAGNSAYYTCDGCDKWFADATGSVEITDKTSVKIPAPGHTAGTEWKSDDTNHWHECTVAGCGVIIESTKSAHTAGEWIVDTPATATTAGTKHKECTVCHRVLETQPIPSTGTELKIIAGDNQIYNKASGSDVTITCNGDFAKFTGIKVDGSVVDSSNYTAVSGSTVLTLKASYLGTLTDGSHTITFVYTDGEANANLTVRTAGSGHIHDYGTEWKSNADNHWHECNCGDKKDEAAHSFKWVVDKEATATKKGSKHEECKICGYKRSAVEIPATGTSTAPTDTTKPNDTTKPGNTNGSEKSPQTGDNS

SEQ ID NO: 84 - protein, 1021 aa, synthetic construct
ASKPDIKVGDYVKMGVYNNASILWRCVSIDNNGPLMLADKIVDTLAYDAKTNDNSNSKSHSRSYKRDDYGSNYWKDSNMRSWLNSTAAEGKVDWLCGNPPKDGYVSGVGAYNEKAGFLNAFSKSEIAAMKTVTQRSLVSHPEYNKGIVDGDANSDLLYYTDISEAVANYDSSYFETTTEKVFLLDVKQANAVWKNLKGYYVAYNNDGMAWPYWLRTPVTDCNHDMRYISSSGQVGRYAPWYSDLGVRPAFYLDSEYFVTTSGSGSQSSPYIGSAPNKQEDDYTISEPAEDANPDWNVSTEQSIQLTLGPWYSNDGKYSNPTIPVYTIQKTRSDTENMVVVVCGEGYTKSQQGKFINDVKRLWQDAMKYEPYRSYADRFNVYALCTASESTFDNGGSTFFDVIVDKYNSPVISNNLHGSQWKNHIFERCIGPEFIEKIHDAHIKKKCDPNTIPSGSEYEPYYYVHDYIAQFAMVVNTKSDFGGAYNNREYGFHYFISPSDSYRASKTFAHEFGHGLLGLGDEYSNGYLLDDKELKSLNLSSVEDPEKIKWRQLLGFRNTYTCRNAYGSKMLVSSYECIMRDTNYQFCEVCRLQGFKRMSQLVKDVDLYVATPEVKEYTGAYSKPSDFTDLETSSYYNYTYNRNDRLLSGNSKSRFNTNMNGKKIELRTVIQNISDKNARQLKFKMWIKHSDGSVATDSSGNPLQTVQTFDIPVWNDKANFWPLGALDHIKSDFNSGLKSCSLIYQIPSDAQLKSGDTVAFQVLDENGNVLADDNTETQRYTTVSIQYGGGGGSESKYGPPCPSCPAPEFLGGPSVFLFPPKPKDTLMISRTPEVTCVVVDVSQEDPEVQFNWYVDGVEVHNAKTKPREEQFNSTYRVVSVLTVLHQDWLNGKEYKCKVSNKGLPSSIEKTISKAKGQPREPQVYTLPPSQEEMTKNQVSLTCLVKGFYPSDIAVEWESNGQPENNYKTTPPVLDSDGSFFLYSRLTVDKSRWQEGNVFSCSVMHEALHNHYTQKSLSLSLGK

SEQ ID NO: 85 - protein, 1377 aa, synthetic construct
ASKPDIKVGDYVKMGVYNNASILWRCVSIDNNGPLMLADKIVDTLAYDAKTNDNSNSKSHSRSYKRDDYGSNYWKDSNMRSWLNSTAAEGKVDWLCGNPPKDGYVSGVGAYNEKAGFLNAFSKSEIAAMKTVTQRSLVSHPEYNKGIVDGDANSDLLYYTDISEAVANYDSSYFETTTEKVFLLDVKQANAVWKNLKGYYVAYNNDGMAWPYWLRTPVTDCNHDMRYISSSGQVGRYAPWYSDLGVRPAFYLDSEYFVTTSGSGSQSSPYIGSAPNKQEDDYTISEPAEDANPDWNVSTEQSIQLTLGPWYSNDGKYSNPTIPVYTIQKTRSDTENMVVVVCGEGYTKSQQGKFINDVKRLWQDAMKYEPYRSYADRFNVYALCTASESTFDNGGSTFFDVIVDKYNSPVISNNLHGSQWKNHIFERCIGPEFIEKIHDAHIKKKCDPNTIPSGSEYEPYYYVHDYIAQFAMVVNTKSDFGGAYNNREYGFHYFISPSDSYRASKTFAHEFGHGLLGLGDEYSNGYLLDDKELKSLNLSSVEDPEKIKWRQLLGFRNTYTCRNAYGSKMLVSSYECIMRDTNYQFCEVCRLQGFKRMSQLVKDVDLYVATPEVKEYTGAYSKPSDFTDLETSSYYNYTYNRNDRLLSGNSKSRFNTNMNGKKIELRTVIQNISDKNARQLKFKMWIKHSDGSVATDSSGNPLQTVQTFDIPVWNDKANFWPLGALDHIKSDFNSGLKSCSLIYQIPSDAQLKSGDTVAFQVLDENGNVLADDNTETQRYTTVSIQYGGGGGSDAHKSEVAHRFKDLGEENFKALVLIAFAQYLQQCPFEDHVKLVNEVTEFAKTCVADESAENCDKSLHTLFGDKLCTVATLRETYGEMADCCAKQEPERNECFLQHKDDNPNLPRLVRPEVDVMCTAFHDNEETFLKKYLYEIARRHPYFYAPELLFFAKRYKAAFTECCQAADKAACLLPKLDELRDEGKASSAKQRLKCASLQKFGERAFKAWAVARLSQRFPKAEFAEVSKLVTDLTKVHTECCHGDLLECADDRADLAKYICENQDSISSKLKECCEKPLLEKSHCIAEVENDEMPADLPSLAADFVESKDVCKNYAEAKDVFLGMFLYEYARRHPDYSVVLLLRLAKTYETTLEKCCAAADPHECYAKVFDEFKPLVEEPQNLIKQNCELFEQLGEYKFQNALLVRYTKKVPQVSTPTLVEVSRNLGKVGSKCCKHPEAKRMPCAEDYLSVVLNQLCVLHEKTPVSDRVTKCCTESLVNRRPCFSALEVDETYVPKEFNAETFTFHADICTLSEKERQIKKQTALVELVKHKPKATKEQLKAVMDDFAAFVEKCCKADDKETCFAEEGKKLVAASQAALGL

SEQ ID NO: 86 - protein, 6 aa, synthetic construct
GGGGGS

SEQ ID NO: 87 - protein, 8 aa, synthetic construct
GGGGGGGS